European Patent Application EP 4 345 454 A2, published April 3, 2024. Title: COMPOSITIONS AND METHODS OF IMPROVING SPECIFICITY IN GENOMIC ENGINEERING USING RNA-GUIDED ENDONUCLEASES. Applicant: DUKE UNIVERSITY. Application EP PCT/US2016/048798, filed August 25, 2016. The sequence listing filed with the application follows.

SEQUENCE LISTING (348 sequences)

SEQ ID NO: 1 - protein, 1368 aa, Streptococcus pyogenes
MDKKYSIGLAIGTNSVGWAVITDEYKVPSKKFKVLGNTDRHSIKKNLIGALLFDSGETAEATRLKRTARRRYTRRKNRICYLQEIFSNEMAKVDDSFFHRLEESFLVEEDKKHERHPIFGNIVDEVAYHEKYPTIYHLRKKLVDSTDKADLRLIYLALAHMIKFRGHFLIEGDLNPDNSDVDKLFIQLVQTYNQLFEENPINASGVDAKAILSARLSKSRRLENLIAQLPGEKKNGLFGNLIALSLGLTPNFKSNFDLAEDAKLQLSKDTYDDDLDNLLAQIGDQYADLFLAAKNLSDAILLSDILRVNTEITKAPLSASMIKRYDEHHQDLTLLKALVRQQLPEKYKEIFFDQSKNGYAGYIDGGASQEEFYKFIKPILEKMDGTEELLVKLNREDLLRKQRTFDNGSIPHQIHLGELHAILRRQEDFYPFLKDNREKIEKILTFRIPYYVGPLARGNSRFAWMTRKSEETITPWNFEEVVDKGASAQSFIERMTNFDKNLPNEKVLPKHSLLYEYFTVYNELTKVKYVTEGMRKPAFLSGEQKKAIVDLLFKTNRKVTVKQLKEDYFKKIECFDSVEISGVEDRFNASLGTYHDLLKIIKDKDFLDNEENEDILEDIVLTLTLFEDREMIEERLKTYAHLFDDKVMKQLKRRRYTGWGRLSRKLINGIRDKQSGKTILDFLKSDGFANRNFMQLIHDDSLTFKEDIQKAQVSGQGDSLHEHIANLAGSPAIKKGILQTVKVVDELVKVMGRHKPENIVIEMARENQTTQKGQKNSRERMKRIEEGIKELGSQILKEHPVENTQLQNEKLYLYYLQNGRDMYVDQELDINRLSDYDVDAIVPQSFLKDDSIDNKVLTRSDKNRGKSDNVPSEEVVKKMKNYWRQLLNAKLITQRKFDNLTKAERGGLSELDKAGFIKRQLVETRQITKHVAQILDSRMNTKYDENDKLIREVKVITLKSKLVSDFRKDFQFYKVREINNYHHAHDAYLNAVVGTALIKKYPKLESEFVYGDYKVYDVRKMIAKSEQEIGKATAKYFFYSNIMNFFKTEITLANGEIRKRPLIETNGETGEIVWDKGRDFATVRKVLSMPQVNIVKKTEVQTGGFSKESILPKRNSDKLIARKKDWDPKKYGGFDSPTVAYSVLVVAKVEKGKSKKLKSVKELLGITIMERSSFEKNPIDFLEAKGYKEVKKDLIIKLPKYSLFELENGRKRMLASAGELQKGNELALPSKYVNFLYLASHYEKLKGSPEDNEQKQLFVEQHKHYLDEIIEQISEFSKRVILADANLDKVLSAYNKHRDKPIREQAENIIHLFTLTNLGAPAAFKYFDTTIDRKRYTSTKEVLDATLIHQSITGLYETRIDLSQLGGD

SEQ ID NO: 2 - protein, 2048 aa, synthetic construct
  REGION 1..2048: note = Description of Artificial Sequence: Syntheticpolypeptide
MDYKDHDGDYKDHDIDYKDDDDKMAPKKKRKVGRGMDKKYSIGLAIGTNSVGWAVITDEYKVPSKKFKVLGNTDRHSIKKNLIGALLFDSGETAEATRLKRTARRRYTRRKNRICYLQEIFSNEMAKVDDSFFHRLEESFLVEEDKKHERHPIFGNIVDEVAYHEKYPTIYHLRKKLVDSTDKADLRLIYLALAHMIKFRGHFLIEGDLNPDNSDVDKLFIQLVQTYNQLFEENPINASGVDAKAILSARLSKSRRLENLIAQLPGEKKNGLFGNLIALSLGLTPNFKSNFDLAEDAKLQLSKDTYDDDLDNLLAQIGDQYADLFLAAKNLSDAILLSDILRVNTEITKAPLSASMIKRYDEHHQDLTLLKALVRQQLPEKYKEIFFDQSKNGYAGYIDGGASQEEFYKFIKPILEKMDGTEELLVKLNREDLLRKQRTFDNGSIPHQIHLGELHAILRRQEDFYPFLKDNREKIEKILTFRIPYYVGPLARGNSRFAWMTRKSEETITPWNFEEVVDKGASAQSFIERMTNFDKNLPNEKVLPKHSLLYEYFTVYNELTKVKYVTEGMRKPAFLSGEQKKAIVDLLFKTNRKVTVKQLKEDYFKKIECFDSVEISGVEDRFNASLGTYHDLLKIIKDKDFLDNEENEDILEDIVLTLTLFEDREMIEERLKTYAHLFDDKVMKQLKRRRYTGWGRLSRKLINGIRDKQSGKTILDFLKSDGFANRNFMQLIHDDSLTFKEDIQKAQVSGQGDSLHEHIANLAGSPAIKKGILQTVKVVDELVKVMGRHKPENIVIEMARENQTTQKGQKNSRERMKRIEEGIKELGSQILKEHPVENTQLQNEKLYLYYLQNGRDMYVDQELDINRLSDYDVDAIVPQSFLKDDSIDNKVLTRSDKNRGKSDNVPSEEVVKKMKNYWRQLLNAKLITQRKFDNLTKAERGGLSELDKAGFIKRQLVETRQITKHVAQILDSRMNTKYDENDKLIREVKVITLKSKLVSDFRKDFQFYKVREINNYHHAHDAYLNAVVGTALIKKYPKLESEFVYGDYKVYDVRKMIAKSEQEIGKATAKYFFYSNIMNFFKTEITLANGEIRKRPLIETNGETGEIVWDKGRDFATVRKVLSMPQVNIVKKTEVQTGGFSKESILPKRNSDKLIARKKDWDPKKYGGFDSPTVAYSVLVVAKVEKGKSKKLKSVKELLGITIMERSSFEKNPIDFLEAKGYKEVKKDLIIKLPKYSLFELENGRKRMLASAGELQKGNELALPSKYVNFLYLASHYEKLKGSPEDNEQKQLFVEQHKHYLDEIIEQISEFSKRVILADANLDKVLSAYNKHRDKPIREQAENIIHLFTLTNLGAPAAFKYFDTTIDRKRYTSTKEVLDATLIHQSITGLYETRIDLSQLGGDPIAGSKASPKKKRKVGRAIFKPEELRQALMPTLEALYRQDPESLPFRQPVDPQLLGIPDYFDIVKSPMDLSTIKRKLDTGQYQEPWQYVDDIWLMFNNAWLYNRKTSRVYKYCSKLSEVFEQEIDPVMQSLGYCCGRKLEFSPQTLCCYGKQLCTIPRDATYYSYQNRYHFCEKCFNEIQGESVSLGDDPSQPQTTINKEQFSKRKNDTLDPELFVECTECGRKMHQICVLHHEIIWPAGFVCDGCLKKSARTRKENKFSAKRLPSTRLGTFLENRVNDFLRRQNHPESGEVTVRVVHASDKTVEVKPGMKARFVDSGEMAESFPYRTKALFAFEEIDGVDLCFFGMHVQEYGSDCPPPNQRRVYISYLDSVHFFRPKCLRTAVYHEILIGYLEYVKKLGYTTGHIWACPPSEGDDYIFHCHPPDQKIPKPKRLQEWYKKMLDKAVSERIVHDYKDIFKQATEDRLTSAKELPYFEGDFWPNVLEESIKELEQEEEERKREENTSNESTDVTKGDSKNAKKKNNKKTSKNKSSLSRGNKKKPGMPNVSNDLSQKLYATMEKHKEVFFVIRLIAGPAANSLPPIVDPDPLIPCDLMDGRDAFLTLARDKHLEFSSLRRAQWSTMCMLVELHTQSQDYPYDVPDYAS

SEQ ID NO: 3 - protein, 1521 aa, synthetic construct
  REGION 1..1521: note = Description of Artificial Sequence: Syntheticpolypeptide
MDYKDHDGDYKDHDIDYKDDDDKMAPKKKRKVGRGMDKKYSIGLAIGTNSVGWAVITDEYKVPSKKFKVLGNTDRHSIKKNLIGALLFDSGETAEATRLKRTARRRYTRRKNRICYLQEIFSNEMAKVDDSFFHRLEESFLVEEDKKHERHPIFGNIVDEVAYHEKYPTIYHLRKKLVDSTDKADLRLIYLALAHMIKFRGHFLIEGDLNPDNSDVDKLFIQLVQTYNQLFEENPINASGVDAKAILSARLSKSRRLENLIAQLPGEKKNGLFGNLIALSLGLTPNFKSNFDLAEDAKLQLSKDTYDDDLDNLLAQIGDQYADLFLAAKNLSDAILLSDILRVNTEITKAPLSASMIKRYDEHHQDLTLLKALVRQQLPEKYKEIFFDQSKNGYAGYIDGGASQEEFYKFIKPILEKMDGTEELLVKLNREDLLRKQRTFDNGSIPHQIHLGELHAILRRQEDFYPFLKDNREKIEKILTFRIPYYVGPLARGNSRFAWMTRKSEETITPWNFEEVVDKGASAQSFIERMTNFDKNLPNEKVLPKHSLLYEYFTVYNELTKVKYVTEGMRKPAFLSGEQKKAIVDLLFKTNRKVTVKQLKEDYFKKIECFDSVEISGVEDRFNASLGTYHDLLKIIKDKDFLDNEENEDILEDIVLTLTLFEDREMIEERLKTYAHLFDDKVMKQLKRRRYTGWGRLSRKLINGIRDKQSGKTILDFLKSDGFANRNFMQLIHDDSLTFKEDIQKAQVSGQGDSLHEHIANLAGSPAIKKGILQTVKVVDELVKVMGRHKPENIVIEMARENQTTQKGQKNSRERMKRIEEGIKELGSQILKEHPVENTQLQNEKLYLYYLQNGRDMYVDQELDINRLSDYDVDAIVPQSFLKDDSIDNKVLTRSDKNRGKSDNVPSEEVVKKMKNYWRQLLNAKLITQRKFDNLTKAERGGLSELDKAGFIKRQLVETRQITKHVAQILDSRMNTKYDENDKLIREVKVITLKSKLVSDFRKDFQFYKVREINNYHHAHDAYLNAVVGTALIKKYPKLESEFVYGDYKVYDVRKMIAKSEQEIGKATAKYFFYSNIMNFFKTEITLANGEIRKRPLIETNGETGEIVWDKGRDFATVRKVLSMPQVNIVKKTEVQTGGFSKESILPKRNSDKLIARKKDWDPKKYGGFDSPTVAYSVLVVAKVEKGKSKKLKSVKELLGITIMERSSFEKNPIDFLEAKGYKEVKKDLIIKLPKYSLFELENGRKRMLASAGELQKGNELALPSKYVNFLYLASHYEKLKGSPEDNEQKQLFVEQHKHYLDEIIEQISEFSKRVILADANLDKVLSAYNKHRDKPIREQAENIIHLFTLTNLGAPAAFKYFDTTIDRKRYTSTKEVLDATLIHQSITGLYETRIDLSQLGGDSRADPKKKRKVASDAKSLTAWSRTLVTFKDVFVDFTREEWKLLDTAQQILYRNVMLENYKNLVSLGYQLTKPDVILRLEKGEEPWLVEREIHQETHPDSETAFEIKSSVPKKKRKVAS

SEQ ID NO: 4 - protein, 617 aa, synthetic construct
  REGION 1..617: note = Description of Artificial Sequence: Syntheticpolypeptide
YKVYDVRKMIAKSEQEIGKATAKYFFYSNIMNFFKTEITLANGEIRKRPLIETNGETGEIVWDKGRDFATVRKVLSMPQVNIVKKTEVQTGGFSKESILPKRNSDKLIARKKDWDPKKYGGFDSPTVAYSVLVVAKVEKGKSKKLKSVKELLGITIMERSSFEKNPIDFLEAKGYKEVKKDLIIKLPKYSLFELENGRKRMLASAGELQKGNELALPSKYVNFLYLASHYEKLKGSPEDNEQKQLFVEQHKHYLDEIIEQISEFSKRVILADANLDKVLSAYNKHRDKPIREQAENIIHLFTLTNLGAPAAFKYFDTTIDRKRYTSTKEVLDATLIHQSITGLYETRIDLSQLGGDPIAGSKASPKKKRKVGRAIFKPEELRQALMPTLEALYRQDPESLPFRQPVDPQLLGIPDYFDIVKSPMDLSTIKRKLDTGQYQEPWQYVDDIWLMFNNAWLYNRKTSRVYKYCSKLSEVFEQEIDPVMQSLGYCCGRKLEFSPQTLCCYGKQLCTIPRDATYYSYQNRYHFCEKCFNEIQGESVSLGDDPSQPQTTINKEQFSKRKNDTLDPELFVECTECGRKMHQICVLHHEIIWPAGFVCDGCLKKSARTRKENKFSA

SEQ ID NO: 5 - protein, 1726 aa, synthetic construct
  REGION 1..1726: note = Description of Artificial Sequence: Syntheticpolypeptide
MAAFKPNPINYILGLAIGIASVGWAMVEIDEDENPICLIDLGVRVFERAEVPKTGDSLAMARRLARSVRRLTRRRAHRLLRARRLLKREGVLQAADFDENGLIKSLPNTPWQLRAAALDRKLTPLEWSAVLLHLIKHRGYLSQRKNEGETADKELGALLKGVADNAHALQTGDFRTPAELALNKFEKESGHIRNQRGDYSHTFSRKDLQAELILLFEKQKEFGNPHVSGGLKEGIETLLMTQRPALSGDAVQKMLGHCTFEPAEPKAAKNTYTAERFIWLTKLNNLRILEQGSERPLTDTERATLMDEPYRKSKLTYAQARKLLGLEDTAFFKGLRYGKDNAEASTLMEMKAYHAISRALEKEGLKDKKSPLNLSPELQDEIGTAFSLFKTDEDITGRLKDRIQPEILEALLKHISFDKFVQISLKALRRIVPLMEQGKRYDEACAEIYGDHYGKKNTEEKIYLPPIPADEIRNPVVLRALSQARKVINGVVRRYGSPARIHIETAREVGKSFKDRKEIEKRQEENRKDREKAAAKFREYFPNFVGEPKSKDILKLRLYEQQHGKCLYSGKEINLGRLNEKGYVEIAAALPFSRTWDDSFNNKVLVLGSEAQNKGNQTPYEYFNGKDNSREWQEFKARVETSRFPRSKKQRILLQKFDEDGFKERNLNDTRYVNRFLCQFVADRMRLTGKGKKRVFASNGQITNLLRGFWGLRKVRAENDRHHALDAVVVACSTVAMQQKITRFVRYKEMNAFDGKTIDKETGEVLHQKTHFPQPWEFFAQEVMIRVFGKPDGKPEFEEADTPEKLRTLLAEKLSSRPEAVHEYVTPLFVSRAPNRKMSGQGHMETVKSAKRLDEGVSVLRVPLTQLKLKDLEKMVNREREPKLYEALKARLEAHKDDPAKAFAEPFYKYDKAGNRTQQVKAVRVEQVQKTGVWVRNHNGIADNATMVRVDVFEKGDKYYLVPIYSWQVAKGILPDRAVVQGKDEEDWQLIDDSFNFKFSLHPNDLVEVITKKARMFGYFASCHRGTGNINIRIHDLDHKIGKNGILEGIGVKTALSFQKYQIDELGKEIRPCRLKKRPPVRSRADPKKKRKVEASGRAIFKPEELRQALMPTLEALYRQDPESLPFRQPVDPQLLGIPDYFDIVKSPMDLSTIKRKLDTGQYQEPWQYVDDIWLMFNNAWLYNRKTSRVYKYCSKLSEVFEQEIDPVMQSLGYCCGRKLEFSPQTLCCYGKQLCTIPRDATYYSYQNRYHFCEKCFNEIQGESVSLGDDPSQPQTTINKEQFSKRKNDTLDPELFVECTECGRKMHQICVLHHEIIWPAGFVCDGCLKKSARTRKENKFSAKRLPSTRLGTFLENRVNDFLRRQNHPESGEVTVRVVHASDKTVEVKPGMKARFVDSGEMAESFPYRTKALFAFEEIDGVDLCFFGMHVQEYGSDCPPPNQRRVYISYLDSVHFFRPKCLRTAVYHEILIGYLEYVKKLGYTTGHIWACPPSEGDDYIFHCHPPDQKIPKPKRLQEWYKKMLDKAVSERIVHDYKDIFKQATEDRLTSAKELPYFEGDFWPNVLEESIKELEQEEEERKREENTSNESTDVTKGDSKNAKKKNNKKTSKNKSSLSRGNKKKPGMPNVSNDLSQKLYATMEKHKEVFFVIRLIAGPAANSLPPIVDPDPLIPCDLMDGRDAFLTLARDKHLEFSSLRRAQWSTMCMLVELHTQSQDYPYDVPDYAS

SEQ ID NO: 6 - RNA, 100 nt, synthetic construct
  misc_feature 1..100: note = Description of Artificial Sequence: Syntheticpolynucleotide
  source 1..100: mol_type = other RNA
ggggccactagggacaggatgttttagagctagaaatagcaagttaaaataaggctagtccgttatcaacttgaaaaagtggcaccgagtcggtgctttt

SEQ ID NO: 7 - RNA, 98 nt, synthetic construct
  misc_feature 1..98: note = Description of Artificial Sequence: Syntheticoligonucleotide
  source 1..98: mol_type = other RNA
ggccactagggacaggatgttttagagctagaaatagcaagttaaaataaggctagtccgttatcaacttgaaaaagtggcaccgagtcggtgctttt

SEQ ID NO: 8 - RNA, 112 nt, synthetic construct
  misc_feature 1..112: note = Description of Artificial Sequence: Syntheticpolynucleotide
  source 1..112: mol_type = other RNA
ggggccccttcgggggccactagggacaggatgttttagagctagaaatagcaagttaaaataaggctagtccgttatcaacttgaaaaagtggcaccgagtcggtgctttt

SEQ ID NO: 9 - RNA, 116 nt, synthetic construct
  misc_feature 1..116: note = Description of Artificial Sequence: Syntheticpolynucleotide
  source 1..116: mol_type = other RNA
ggtagtggccccttcgggggccactagggacaggatgttttagagctagaaatagcaagttaaaataaggctagtccgttatcaacttgaaaaagtggcaccgagtcggtgctttt

SEQ ID NO: 10 - DNA, 1198 bp, synthetic construct
  misc_feature 1..1198: note = Description of Artificial Sequence: Syntheticpolynucleotide
  source 1..1198: mol_type = other DNA
ccaggatcagtgaaacgcaccagacagccgcgtcagagcagctcaggttctgggagagggtagcgcagggtggccactgagaaccgggcaggtcacgcatcccccccttccctcccaccccctgccaagctctccctcccaggatcctctctggctccatcgtaagcaaaccttagaggttctggcaaggagagagatggctccaggaaatgggggtgtgtcaccagataaggaatctgcctaacaggaggtgggggttagacccaatatcaggagactaggaaggaggaggcctaaggatggggcttttctgtcaccaatcctgtccctagtggccccactgtggggtggaggggacagataaaagtacccagaaccagagccacattaaccggccctgggaatataaggtggtcccagctcggggacacaggatccctggaggcagcaaacatgctgtcctgaagtggacataggggcccgggttggaggaagaagactagctgagctctcggacccctggaagatgccatgacagggggctggaagagctagcacagactagagaggtaaggggggtaggggagctgcccaaatgaaaggagtgagaggtgacccggaatccacaggagaacggggtgtccaggcaaagaaagcaagaggatggagaggtggctaaagccagggagacggggtactttggggttgtccagaaaaacggtgatgatgcaggcctacaagaaggggaggcgggacgcaagggagacatccgtcggagaaggccatcctaagaaacgagagatggcacaggccccagaaggagaaggaaaagggaacccagcgagtgaagacggcatggggttgggtgagggaggagagatgcccggagaggacccagacacggggaggatccgctcagaggacatcacgtggtgcagcgccgagaaggaagtgctccggaaagagcatccttgggcagcaacacagcagagagcaaggggaagagggagtggaggaagacggaacctgaaggaggcggcagggaaggatctgggccagccgtagaggtgacccaggccacaagctgcagacagaaagcggcacaggcccaggggagagaatgcaggtcagagaaagcaggacctgcctgggaaggggaaacagtgggccagaggcggcgcagaagccagtagagctc

SEQ ID NO: 11 - DNA, 986 bp, synthetic construct
  misc_feature 1..986: note = Description of Artificial Sequence: Syntheticpolynucleotide
  source 1..986: mol_type = other DNA
catgacgtgcagcaagcgcgctgacgcagctaattttatctatgtgcttcgtcatacgtgatgcatatactctctgctagctgactcattcagctgtactcactcgctgttgagtctcatacagcgcgagatcaaatgagtcatccaatcctgtccctagtggcccctatcgtgacactgcactgcagcgtacgcgacagagctagacttcgtttcaatacagactagctactgcgtctgcagagcgctctcttgtcacttacatcgaagtcaacgcgctcgcgttcagagatcttctccaatcctactttcgacaattttcgctctcagcgtttgtgtctgtgcgcgcacacagtctgtgcttcgcttgcaactaacgtagcgcttcagcgcatcgtcaaagagcgaaagagtcacagtgtctgtgttcacgtctctatctttctagttctccaatcctgtcccaaaattgtcgaagacagagtttcgcgaattcgcagcagcgcgatctctgctcactgcaatctctgactgctgcttttaagcaattctcgcagctcagcatgagtacttgcgattacagcagtgctcgccaatcctgtccctagtgattttgcagcgtcagcagagctgatgagatgcagttcagcatcgcagacgagcagcacgaagcgagcatctgtagaaaatcgatcgacgcgcacttgcagagacaccaaaaattgtcgaaagtgaagccttgtctctcgttcgcatcaagacacgctatttctgtctcttaaatgtttcaaaaacacatcatgtcttcttcgtgcgagttcgatgcgcgtgtgcgagaccacgcctgtccctagtggcccctgactctctgtgcattttgagctgcgaaagtaaagatatcgttcattgcagagacagagctagtactagtctcagttcttgcactatgctctcgatgtctctcttagtgattcagcgcatcgtcg

SEQ ID NO: 12 - DNA, 1078 bp, synthetic construct
  misc_feature 1..1078: note = Description of Artificial Sequence: Syntheticpolynucleotide
  source 1..1078: mol_type = other DNA
gacctgcaggcatgcaagcttgggctagcggagagtcagttcgcggtactggaggaggcggcgcaacgtcgccagctgtctgcacaggagaaatccctgctggcgcataaagatgagacgctggagtacaaacgccagctggctgcacttggcgacaaggttacgtatcaggagcgcctgaacgcgctggcgcagcaggcggataaattcgcacagcagcaacgggcaaaacgggccgccattgatgcgaaaagccgggggctgactgaccggcaggcagaacgggaagccacggaacagcgcctgaaggaacagtatggcgataatccgctggcgctgaataacgtcatgtcagagcagaaaaagacctgggcggctgaagaccagcttcgcgggaactggatggcaggcctgaagtccggctggccatgggctgaggccagctgaggtaccgctgaggattgctgaggtgtacagacgctcaagtcagaggtggcgagagctcccggagtggctcacagtcggtggtccggcagtacaatggattaccgtaagacggaaatcactcccgggtatatgaaagagacgaccactgccagggacgaaagtgcaatgcggcatacctcagtggcgtggagtgcaggtatacagattaatccggcagcgtccgtcgttgttgatattgcttatgaaggctccggcagtggcgactggcgtactgacggattcatcgttggggtcggttataaattctgattagccaggtaacacagtgttatgacagcccgccggaaccggtgggcttttttgtggggtgaatatggcagtaaagatttcaggagtcctgaaagacggcacaggaaaaccggtacagaactgcaccattcagctgaaagccagacgtaacagcaccacggtggtggtgaacacggtgggctcagagaatccggatgaagccgggcgttacagcatggatgtggagtacggtcagtacagtgtcatcctgcaggttgacggttttccaccatcgcacgccgggaccatcaccgtgtatgaagattcacaaccggggacgctg

SEQ ID NO: 13 - DNA, 20 bp, synthetic construct
  misc_feature 1..20: note = Description of Artificial Sequence: Syntheticoligonucleotide
  source 1..20: mol_type = other DNA
ttcttcttctgctcggactc

SEQ ID NO: 14 - DNA, 20 bp, synthetic construct
  misc_feature 1..20: note = Description of Artificial Sequence: Syntheticoligonucleotide
  source 1..20: mol_type = other DNA
ttcttcttctgctcggactc

SEQ ID NO: 15 - DNA, 20 bp, synthetic construct
  misc_feature 1..20: note = Description of Artificial Sequence: Syntheticoligonucleotide
  source 1..20: mol_type = other DNA
ttcttcttctgctcggactc

SEQ ID NO: 16 - DNA, 20 bp, synthetic construct
  misc_feature 1..20: note = Description of Artificial Sequence: Syntheticoligonucleotide
  source 1..20: mol_type = other DNA
ttcttcttctgctcggactc

SEQ ID NO: 17 - DNA, 20 bp, synthetic construct
  misc_feature 1..20: note = Description of Artificial Sequence: Syntheticoligonucleotide
  source 1..20: mol_type = other DNA
ttcttcttctgctcggactc

SEQ ID NO: 18 - DNA, 20 bp, synthetic construct
  misc_feature 1..20: note = Description of Artificial Sequence: Syntheticoligonucleotide
  source 1..20: mol_type = other DNA
ttcttcttctgctcggactc

SEQ ID NO: 19 - DNA, 20 bp, synthetic construct
  misc_feature 1..20: note = Description of Artificial Sequence: Syntheticoligonucleotide
  source 1..20: mol_type = other DNA
ttcttcttctgctcggactc

SEQ ID NO: 20 - DNA, 20 bp, synthetic construct
  misc_feature 1..20: note = Description of Artificial Sequence: Syntheticoligonucleotide
  source 1..20: mol_type = other DNA
ttcttcttctgctcggactc

SEQ ID NO: 21 - DNA, 20 bp, synthetic construct
  misc_feature 1..20: note = Description of Artificial Sequence: Syntheticoligonucleotide
  source 1..20: mol_type = other DNA
ttcttcttctgctcggactc

SEQ ID NO: 22 - DNA, 20 bp, synthetic construct
  misc_feature 1..20: note = Description of Artificial Sequence: Syntheticoligonucleotide
  source 1..20: mol_type = other DNA
ttcttcttctgctcggactc

SEQ ID NO: 23 - DNA, 20 bp, synthetic construct
  misc_feature 1..20: note = Description of Artificial Sequence: Syntheticoligonucleotide
  source 1..20: mol_type = other DNA
ttcttcttctgctcggactc

SEQ ID NO: 24 - DNA, 20 bp, synthetic construct
  misc_feature 1..20: note = Description of Artificial Sequence: Syntheticoligonucleotide
  source 1..20: mol_type = other DNA
ttcttcttctgctcggactc

SEQ ID NO: 25 - DNA, 20 bp, synthetic construct
  misc_feature 1..20: note = Description of Artificial Sequence: Syntheticoligonucleotide
  source 1..20: mol_type = other DNA
ttcttcttctgctcggactc

SEQ ID NO: 26 - DNA, 20 bp, synthetic construct
  misc_feature 1..20: note = Description of Artificial Sequence: Syntheticoligonucleotide
  source 1..20: mol_type = other DNA
ttcttcttctgctcggactc

SEQ ID NO: 27 - DNA, 20 bp, synthetic construct
  misc_feature 1..20: note = Description of Artificial Sequence: Syntheticoligonucleotide
  source 1..20: mol_type = other DNA
ttcttcttctgctcggactc

SEQ ID NO: 28 - DNA, 20 bp, synthetic construct
  misc_feature 1..20: note = Description of Artificial Sequence: Syntheticoligonucleotide
  source 1..20: mol_type = other DNA
ttcttcttctgctcggactc

SEQ ID NO: 29 - DNA, 20 bp, synthetic construct
  misc_feature 1..20: note = Description of Artificial Sequence: Syntheticoligonucleotide
  source 1..20: mol_type = other DNA
ttcttcttctgctcggactc

SEQ ID NO: 30 - DNA, 20 bp, synthetic construct
  misc_feature 1..20: note = Description of Artificial Sequence: Syntheticoligonucleotide
  source 1..20: mol_type = other DNA
ttcttcttctgctcggactc

SEQ ID NO: 31 - DNA, 20 bp, synthetic construct
  misc_feature 1..20: note = Description of Artificial Sequence: Syntheticoligonucleotide
  source 1..20: mol_type = other DNA
ttcttcttctgctcggactc

SEQ ID NO: 32 - DNA, 20 bp, synthetic construct
  misc_feature 1..20: note = Description of Artificial Sequence: Syntheticoligonucleotide
  source 1..20: mol_type = other DNA
ttcttcttctgctcggactc

SEQ ID NO: 33 - DNA, 20 bp, synthetic construct
  misc_feature 1..20: note = Description of Artificial Sequence: Syntheticoligonucleotide
  source 1..20: mol_type = other DNA
ccctagtcattggaggtgac

SEQ ID NO: 34 - DNA, 20 bp, synthetic construct
  misc_feature 1..20: note = Description of Artificial Sequence: Syntheticoligonucleotide
  source 1..20: mol_type = other DNA
ccctagtcattggaggtgac

SEQ ID NO: 35 - DNA, 20 bp, synthetic construct
  misc_feature 1..20: note = Description of Artificial Sequence: Syntheticoligonucleotide
  source 1..20: mol_type = other DNA
ccctagtcattggaggtgac

SEQ ID NO: 36 - DNA, 20 bp, synthetic construct
  misc_feature 1..20: note = Description of Artificial Sequence: Syntheticoligonucleotide
  source 1..20: mol_type = other DNA
ccctagtcattggaggtgac

SEQ ID NO: 37 - DNA, 20 bp, synthetic construct
  misc_feature 1..20: note = Description of Artificial Sequence: Syntheticoligonucleotide
  source 1..20: mol_type = other DNA
ccctagtcattggaggtgac

SEQ ID NO: 38 - DNA, 20 bp, synthetic construct
  misc_feature 1..20: note = Description of Artificial Sequence: Syntheticoligonucleotide
  source 1..20: mol_type = other DNA
ccctagtcattggaggtgac

SEQ ID NO: 39 - DNA, 20 bp, synthetic construct
  misc_feature 1..20: note = Description of Artificial Sequence: Syntheticoligonucleotide
  source 1..20: mol_type = other DNA
ccctagtcattggaggtgac

SEQ ID NO: 40 - DNA, 20 bp, synthetic construct
  misc_feature 1..20: note = Description of Artificial Sequence: Syntheticoligonucleotide
  source 1..20: mol_type = other DNA
ccctagtcattggaggtgac

SEQ ID NO: 41 - DNA, 20 bp, synthetic construct
  misc_feature 1..20: note = Description of Artificial Sequence: Syntheticoligonucleotide
  source 1..20: mol_type = other DNA
ccctagtcattggaggtgac

SEQ ID NO: 42 - DNA, 20 bp, synthetic construct
  misc_feature 1..20: note = Description of Artificial Sequence: Syntheticoligonucleotide
  source 1..20: mol_type = other DNA
ccctagtcattggaggtgac

SEQ ID NO: 43 - DNA, 20 bp, synthetic construct
  misc_feature 1..20: note = Description of Artificial Sequence: Syntheticoligonucleotide
  source 1..20: mol_type = other DNA
atggggaggacatcgatgtc

SEQ ID NO: 44 - DNA, 20 bp, synthetic construct
  misc_feature 1..20: note = Description of Artificial Sequence: Syntheticoligonucleotide
  source 1..20: mol_type = other DNA
atggggaggacatcgatgtc

SEQ ID NO: 45 - DNA, 20 bp, synthetic construct
  misc_feature 1..20: note = Description of Artificial Sequence: Syntheticoligonucleotide
  source 1..20: mol_type = other DNA
atggggaggacatcgatgtc

SEQ ID NO: 46 - DNA, 20 bp, synthetic construct
  misc_feature 1..20: note = Description of Artificial Sequence: Syntheticoligonucleotide
  source 1..20: mol_type = other DNA
atggggaggacatcgatgtc

SEQ ID NO: 47 - DNA, 20 bp, synthetic construct
  misc_feature 1..20: note = Description of Artificial Sequence: Syntheticoligonucleotide
  source 1..20: mol_type = other DNA
atggggaggacatcgatgtc

SEQ ID NO: 48 - DNA, 20 bp, synthetic construct
  misc_feature 1..20: note = Description of Artificial Sequence: Syntheticoligonucleotide
  source 1..20: mol_type = other DNA
atggggaggacatcgatgtc

SEQ ID NO: 49 - DNA, 20 bp, synthetic construct
  misc_feature 1..20: note = Description of Artificial Sequence: Syntheticoligonucleotide
  source 1..20: mol_type = other DNA
atggggaggacatcgatgtc

SEQ ID NO: 50 - DNA, 20 bp, synthetic construct
  misc_feature 1..20: note = Description of Artificial Sequence: Syntheticoligonucleotide
  source 1..20: mol_type = other DNA
atggggaggacatcgatgtc

SEQ ID NO: 51 - DNA, 20 bp, synthetic construct
  misc_feature 1..20: note = Description of Artificial Sequence: Syntheticoligonucleotide
  source 1..20: mol_type = other DNA
atggggaggacatcgatgtc

SEQ ID NO: 52 - DNA, 20 bp, synthetic construct
  misc_feature 1..20: note = Description of Artificial Sequence: Syntheticoligonucleotide
  source 1..20: mol_type = other DNA
atggggaggacatcgatgtc

SEQ ID NO: 53 - DNA, 20 bp, synthetic construct
  misc_feature 1..20: note = Description of Artificial Sequence: Syntheticoligonucleotide
  source 1..20: mol_type = other DNA
atcacatcaaccggtggcgc

SEQ ID NO: 54 - DNA, 20 bp, synthetic construct
  misc_feature 1..20: note = Description of Artificial Sequence: Syntheticoligonucleotide
  source 1..20: mol_type = other DNA
atcacatcaaccggtggcgc

SEQ ID NO: 55 - DNA, 20 bp, synthetic construct
  misc_feature 1..20: note = Description of Artificial Sequence: Syntheticoligonucleotide
  source 1..20: mol_type = other DNA
atcacatcaaccggtggcgc

SEQ ID NO: 56 - DNA, 20 bp, synthetic construct
  misc_feature 1..20: note = Description of Artificial Sequence: Syntheticoligonucleotide
  source 1..20: mol_type = other DNA
atcacatcaaccggtggcgc

SEQ ID NO: 57 - DNA, 20 bp, synthetic construct
  misc_feature 1..20: note = Description of Artificial Sequence: Syntheticoligonucleotide
  source 1..20: mol_type = other DNA
atcacatcaaccggtggcgc

SEQ ID NO: 58 - DNA, 20 bp, synthetic construct
  misc_feature 1..20: note = Description of Artificial Sequence: Syntheticoligonucleotide
  source 1..20: mol_type = other DNA
atcacatcaaccggtggcgc

SEQ ID NO: 59 - DNA, 20 bp, synthetic construct
  misc_feature 1..20: note = Description of Artificial Sequence: Syntheticoligonucleotide
  source 1..20: mol_type = other DNA
atcacatcaaccggtggcgc

SEQ ID NO: 60 - DNA, 20 bp, synthetic construct
  misc_feature 1..20: note = Description of Artificial Sequence: Syntheticoligonucleotide
  source 1..20: mol_type = other DNA
atcacatcaaccggtggcgc

SEQ ID NO: 61 - DNA, 20 bp, synthetic construct
  misc_feature 1..20: note = Description of Artificial Sequence: Syntheticoligonucleotide
  source 1..20: mol_type = other DNA
atcacatcaaccggtggcgc

SEQ ID NO: 62 - DNA, 20 bp, synthetic construct
  misc_feature 1..20: note = Description of Artificial Sequence: Syntheticoligonucleotide
  source 1..20: mol_type = other DNA
atcacatcaaccggtggcgc

SEQ ID NO: 63 - DNA, 20 bp, synthetic construct
  misc_feature 1..20: note = Description of Artificial Sequence: Syntheticoligonucleotide
  source 1..20: mol_type = other DNA
gagtttctcatctgtgcccc

SEQ ID NO: 64 - DNA, 20 bp, synthetic construct
  misc_feature 1..20: note = Description of Artificial Sequence: Syntheticoligonucleotide
  source 1..20: mol_type = other DNA
ccagcttctgccgtttgtac

SEQ ID NO: 65 - DNA, 20 bp, synthetic construct
  misc_feature 1..20: note = Description of Artificial Sequence: Syntheticoligonucleotide
  source 1..20: mol_type = other DNA
ccagcttctgccgtttgtac

SEQ ID NO: 66 - DNA, 20 bp, synthetic construct
  misc_feature 1..20: note = Description of Artificial Sequence: Syntheticoligonucleotide
  source 1..20: mol_type = other DNA
ccagcttctgccgtttgtac

SEQ ID NO: 67 - DNA, 20 bp, synthetic construct
  misc_feature 1..20: note = Description of Artificial Sequence: Syntheticoligonucleotide
  source 1..20: mol_type = other DNA
ttcctcctccagcttctgcc

SEQ ID NO: 68 - DNA, 20 bp, synthetic construct
  misc_feature 1..20: note = Description of Artificial Sequence: Syntheticoligonucleotide
  source 1..20: mol_type = other DNA
ttcctcctccagcttctgcc

SEQ ID NO: 69 - DNA, 20 bp, synthetic construct
  misc_feature 1..20: note = Description of Artificial Sequence: Syntheticoligonucleotide
  source 1..20: mol_type = other DNA
ttcctcctccagcttctgcc

SEQ ID NO: 70 - DNA, 20 bp, synthetic construct
  misc_feature 1..20: note = Description of Artificial Sequence: Syntheticoligonucleotide
  source 1..20: mol_type = other DNA
ttcctcctccagcttctgcc

SEQ ID NO: 71 - DNA, 20 bp, synthetic construct
  misc_feature 1..20: note = Description of Artificial Sequence: Syntheticoligonucleotide
  source 1..20: mol_type = other DNA
ttcctcctccagcttctgcc

SEQ ID NO: 72 - DNA, 20 bp, synthetic construct
  misc_feature 1..20: note = Description of Artificial Sequence: Syntheticoligonucleotide
  source 1..20: mol_type = other DNA
ccggttgatgtgatgggagc

SEQ ID NO: 73 - DNA, 20 bp, synthetic construct
  misc_feature 1..20: note = Description of Artificial Sequence: Syntheticoligonucleotide
  source 1..20: mol_type = other DNA
ccggttgatgtgatgggagc

SEQ ID NO: 74 - DNA, 20 bp, synthetic construct
  misc_feature 1..20: note = Description of Artificial Sequence: Syntheticoligonucleotide
  source 1..20: mol_type = other DNA
ccggttgatgtgatgggagc

SEQ ID NO: 75 - DNA, 20 bp, synthetic construct
  misc_feature 1..20: note = Description of Artificial Sequence: Syntheticoligonucleotide
  source 1..20: mol_type = other DNA
ccggttgatgtgatgggagc

SEQ ID NO: 76 - DNA, 20 bp, synthetic construct
  misc_feature 1..20: note = Description of Artificial Sequence: Syntheticoligonucleotide
  source 1..20: mol_type = other DNA
gcagcaagcagcactctgcc

SEQ ID NO: 77 - DNA, 20 bp, synthetic construct
  misc_feature 1..20: note = Description of Artificial Sequence: Syntheticoligonucleotide
  source 1..20: mol_type = other DNA
gcagcaagcagcactctgcc

SEQ ID NO: 78 - DNA, 20 bp, synthetic construct
  misc_feature 1..20: note = Description of Artificial Sequence: Syntheticoligonucleotide
  source 1..20: mol_type = other DNA
gcttgggcccacgcaggggc

SEQ ID NO: 79 - DNA, 20 bp, synthetic construct
  misc_feature 1..20: note = Description of Artificial Sequence: Syntheticoligonucleotide
  source 1..20: mol_type = other DNA
gcttgggcccacgcaggggc

SEQ ID NO: 80 - DNA, 20 bp, synthetic construct
  misc_feature 1..20: note = Description of Artificial Sequence: Syntheticoligonucleotide
  source 1..20: mol_type = other DNA
gcttcgtggcaatgcgccac

SEQ ID NO: 81 - DNA, 20 bp, synthetic construct
  misc_feature 1..20: note = Description of Artificial Sequence: Syntheticoligonucleotide
  source 1..20: mol_type = other DNA
gcttgggcccacgcaggggc

SEQ ID NO: 82 - DNA, 20 bp, synthetic construct
  misc_feature 1..20: note = Description of Artificial Sequence: Syntheticoligonucleotide
  source 1..20: mol_type = other DNA
aagctggactctggccactc

SEQ ID NO: 83 - DNA, 20 bp, synthetic construct
  misc_feature 1..20: note = Description of Artificial Sequence: Syntheticoligonucleotide
  source 1..20: mol_type = other DNA
ttcttcttctgctcggactc

SEQ ID NO: 84 - DNA, 20 bp, synthetic construct
  misc_feature 1..20: note = Description of Artificial Sequence: Syntheticoligonucleotide
  source 1..20: mol_type = other DNA
ttcttcttctgctcggactc

SEQ ID NO: 85 - DNA, 20 bp, synthetic construct
  misc_feature 1..20: note = Description of Artificial Sequence: Syntheticoligonucleotide
  source 1..20: mol_type = other DNA
ttcttcttctgctcggactc

SEQ ID NO: 86 - DNA, 20 bp, synthetic construct
  misc_feature 1..20: note = Description of Artificial Sequence: Syntheticoligonucleotide
  source 1..20: mol_type = other DNA
gagtttctcatctgtgcccc

SEQ ID NO: 87 - DNA, 20 bp, synthetic construct
  misc_feature 1..20: note = Description of Artificial Sequence: Syntheticoligonucleotide
  source 1..20: mol_type = other DNA
ttcctcctccagcttctgcc

SEQ ID NO: 88 - DNA, 20 bp, synthetic construct
  misc_feature 1..20: note = Description of Artificial Sequence: Syntheticoligonucleotide
  source 1..20: mol_type = other DNA
ttcctcctccagcttctgcc

SEQ ID NO: 89 - DNA, 20 bp, synthetic construct
  misc_feature 1..20: note = Description of Artificial Sequence: Syntheticoligonucleotide
  source 1..20: mol_type = other DNA
agcagaagaagaagggctcc

SEQ ID NO: 90 - DNA, 20 bp, synthetic construct
  misc_feature 1..20: note = Description of Artificial Sequence: Syntheticoligonucleotide
  source 1..20: mol_type = other DNA
aagctggactctggccactc

SEQ ID NO: 91 - DNA, 20 bp, synthetic construct
  misc_feature 1..20: note = Description of Artificial Sequence: Syntheticoligonucleotide
  source 1..20: mol_type = other DNA
ccctagtcattggaggtgac

SEQ ID NO: 92 - DNA, 20 bp, synthetic construct
  misc_feature 1..20: note = Description of Artificial Sequence: Syntheticoligonucleotide
  source 1..20: mol_type = other DNA
ccctagtcattggaggtgac

SEQ ID NO: 93 - DNA, 20 bp, synthetic construct
  misc_feature 1..20: note = Description of Artificial Sequence: Syntheticoligonucleotide
  source 1..20: mol_type = other DNA
ccctagtcattggaggtgac

SEQ ID NO: 94 - DNA, 20 bp, synthetic construct
  misc_feature 1..20: note = Description of Artificial Sequence: Syntheticoligonucleotide
  source 1..20: mol_type = other DNA
ccctagtcattggaggtgac

SEQ ID NO: 95 - DNA, 20 bp, synthetic construct
  misc_feature 1..20: note = Description of Artificial Sequence: Syntheticoligonucleotide
  source 1..20: mol_type = other DNA
ccctagtcattggaggtgac

SEQ ID NO: 96 - DNA, 20 bp, synthetic construct
  misc_feature 1..20: note = Description of Artificial Sequence: Syntheticoligonucleotide
  source 1..20: mol_type = other DNA
ccctagtcattggaggtgac

SEQ ID NO: 97 - DNA, 20 bp, synthetic construct
  misc_feature 1..20: note = Description of Artificial Sequence: Syntheticoligonucleotide
  source 1..20: mol_type = other DNA
ccctagtcattggaggtgac

SEQ ID NO: 98 - DNA, 20 bp, synthetic construct
  misc_feature 1..20: note = Description of Artificial Sequence: Syntheticoligonucleotide
  source 1..20: mol_type = other DNA
ccctagtcattggaggtgac

SEQ ID NO: 99 - DNA, 20 bp, synthetic construct
  misc_feature 1..20: note = Description of Artificial Sequence: Syntheticoligonucleotide
  source 1..20: mol_type = other DNA
ccctagtcattggaggtgac

SEQ ID NO: 100 - DNA, 20 bp, synthetic construct
  misc_feature 1..20: note = Description of Artificial Sequence: Syntheticoligonucleotide
  source 1..20: mol_type = other DNA
ccctagtcattggaggtgac

SEQ ID NO: 101 - DNA, 20 bp, synthetic construct
  misc_feature 1..20: note = Description of Artificial Sequence: Syntheticoligonucleotide
  source 1..20: mol_type = other DNA
atggggaggacatcgatgtc

SEQ ID NO: 102 - DNA, 20 bp, synthetic construct
  misc_feature 1..20: note = Description of Artificial Sequence: Syntheticoligonucleotide
  source 1..20: mol_type = other DNA
atggggaggacatcgatgtc

SEQ ID NO: 103 - DNA, 20 bp, synthetic construct
  misc_feature 1..20: note = Description of Artificial Sequence: Syntheticoligonucleotide
  source 1..20: mol_type = other DNA
atggggaggacatcgatgtc

SEQ ID NO: 104 - DNA, 20 bp, synthetic construct
  misc_feature 1..20: note = Description of Artificial Sequence: Syntheticoligonucleotide
  source 1..20: mol_type = other DNA
atggggaggacatcgatgtc

SEQ ID NO: 105 - DNA, 20 bp, synthetic construct
  misc_feature 1..20: note = Description of Artificial Sequence: Syntheticoligonucleotide
  source 1..20: mol_type = other DNA
atggggaggacatcgatgtc

SEQ ID NO: 106 - DNA, 20 bp, synthetic construct
  misc_feature 1..20: note = Description of Artificial Sequence: Syntheticoligonucleotide
  source 1..20: mol_type = other DNA
atggggaggacatcgatgtc

SEQ ID NO: 107 - DNA, 20 bp, synthetic construct
  misc_feature 1..20: note = Description of Artificial Sequence: Syntheticoligonucleotide
  source 1..20: mol_type = other DNA
atggggaggacatcgatgtc

SEQ ID NO: 108 - DNA, 20 bp, synthetic construct
  misc_feature 1..20: note = Description of Artificial Sequence: Syntheticoligonucleotide
  source 1..20: mol_type = other DNA
atggggaggacatcgatgtc

SEQ ID NO: 109 - DNA, 20 bp, synthetic construct
  misc_feature 1..20: note = Description of Artificial Sequence: Syntheticoligonucleotide
  source 1..20: mol_type = other DNA
atggggaggacatcgatgtc

SEQ ID NO: 110 - DNA, 20 bp, synthetic construct
  misc_feature 1..20: note = Description of Artificial Sequence: Syntheticoligonucleotide
  source 1..20: mol_type = other DNA
atggggaggacatcgatgtc

SEQ ID NO: 111 - DNA, 20 bp, synthetic construct
  misc_feature 1..20: note = Description of Artificial Sequence: Syntheticoligonucleotide
  source 1..20: mol_type = other DNA
atcacatcaaccggtggcgc

SEQ ID NO: 112 - DNA, 20 bp, synthetic construct
  misc_feature 1..20: note = Description of Artificial Sequence: Syntheticoligonucleotide
  source 1..20: mol_type = other DNA
atcacatcaaccggtggcgc

SEQ ID NO: 113 - DNA, 20 bp, synthetic construct
  misc_feature 1..20: note = Description of Artificial Sequence: Syntheticoligonucleotide
  source 1..20: mol_type = other DNA
atcacatcaaccggtggcgc

SEQ ID NO: 114 - DNA, 20 bp, synthetic construct
  misc_feature 1..20: note = Description of Artificial Sequence: Syntheticoligonucleotide
  source 1..20: mol_type = other DNA
atcacatcaaccggtggcgc

SEQ ID NO: 115 - DNA, 20 bp, synthetic construct
  misc_feature 1..20: note = Description of Artificial Sequence: Syntheticoligonucleotide
  source 1..20: mol_type = other DNA
atcacatcaaccggtggcgc

SEQ ID NO: 116 - DNA, 20 bp, synthetic construct
  misc_feature 1..20: note = Description of Artificial Sequence: Syntheticoligonucleotide
  source 1..20: mol_type = other DNA
atcacatcaaccggtggcgc

SEQ ID NO: 117 - DNA, 20 bp, synthetic construct
  misc_feature 1..20: note = Description of Artificial Sequence: Syntheticoligonucleotide
  source 1..20: mol_type = other DNA
atcacatcaaccggtggcgc

SEQ ID NO: 118 - DNA, 20 bp, synthetic construct
  misc_feature 1..20: note = Description of Artificial Sequence: Syntheticoligonucleotide
  source 1..20: mol_type = other DNA
atcacatcaaccggtggcgc

SEQ ID NO: 119 - DNA, 20 bp, synthetic construct
  misc_feature 1..20: note = Description of Artificial Sequence: Syntheticoligonucleotide
  source 1..20: mol_type = other DNA
atcacatcaaccggtggcgc

SEQ ID NO: 120 - DNA, 20 bp, synthetic construct
  misc_feature 1..20: note = Description of Artificial Sequence: Syntheticoligonucleotide
  source 1..20: mol_type = other DNA
atcacatcaaccggtggcgc

SEQ ID NO: 121 - DNA, 20 bp, synthetic construct
  misc_feature 1..20: note = Description of Artificial Sequence: Syntheticoligonucleotide
  source 1..20: mol_type = other DNA
gagtttctcatctgtgcccc

SEQ ID NO: 122 - DNA, 20 bp, synthetic construct
  misc_feature 1..20: note = Description of Artificial Sequence: Syntheticoligonucleotide
  source 1..20: mol_type = other DNA
ccagcttctgccgtttgtac

SEQ ID NO: 123 - DNA, 20 bp, synthetic construct
  misc_feature 1..20: note = Description of Artificial Sequence: Syntheticoligonucleotide
  source 1..20: mol_type = other DNA
ccagcttctgccgtttgtac

SEQ ID NO: 124 - DNA, 20 bp, synthetic construct
  misc_feature 1..20: note = Description of Artificial Sequence: Syntheticoligonucleotide
  source 1..20: mol_type = other DNA
ccagcttctgccgtttgtac

SEQ ID NO: 125 - DNA, 20 bp, synthetic construct
  misc_feature 1..20: note = Description of Artificial Sequence: Syntheticoligonucleotide
  source 1..20: mol_type = other DNA
ttcctcctccagcttctgcc

SEQ ID NO: 126 - DNA, 20 bp, synthetic construct
  misc_feature 1..20: note = Description of Artificial Sequence: Syntheticoligonucleotide
  source 1..20: mol_type = other DNA
ttcctcctccagcttctgcc

SEQ ID NO: 127 - DNA, 20 bp, synthetic construct
  misc_feature 1..20: note = Description of Artificial Sequence: Syntheticoligonucleotide
  source 1..20: mol_type = other DNA
ttcctcctccagcttctgcc

SEQ ID NO: 128 - DNA, 20 bp, synthetic construct
  misc_feature 1..20: note = Description of Artificial Sequence: Syntheticoligonucleotide
  source 1..20: mol_type = other DNA
ttcctcctccagcttctgcc

SEQ ID NO: 129 - DNA, 20 bp, synthetic construct
  misc_feature 1..20: note = Description of Artificial Sequence: Syntheticoligonucleotide
  source 1..20: mol_type = other DNA
ttcctcctccagcttctgcc

SEQ ID NO: 130 - DNA, 20 bp, synthetic construct
  misc_feature 1..20: note = Description of Artificial Sequence: Syntheticoligonucleotide
  source 1..20: mol_type = other DNA
ccggttgatgtgatgggagc

SEQ ID NO: 131 - DNA, 20 bp, synthetic construct
  misc_feature 1..20: note = Description of Artificial Sequence: Syntheticoligonucleotide
  source 1..20: mol_type = other DNA
ccggttgatgtgatgggagc

SEQ ID NO: 132 - DNA, 20 bp, synthetic construct
  misc_feature 1..20: note = Description of Artificial Sequence: Syntheticoligonucleotide
  source 1..20: mol_type = other DNA
ccggttgatgtgatgggagc

SEQ ID NO: 133 - DNA, 20 bp, synthetic construct
  misc_feature 1..20: note = Description of Artificial Sequence: Syntheticoligonucleotide
  source 1..20: mol_type = other DNA
ccggttgatgtgatgggagc

SEQ ID NO: 134 - DNA, 20 bp, synthetic construct
  misc_feature 1..20: note = Description of Artificial Sequence: Syntheticoligonucleotide
  source 1..20: mol_type = other DNA
gcagcaagcagcactctgcc

SEQ ID NO: 135 - DNA, 20 bp, synthetic construct
  misc_feature 1..20: note = Description of Artificial Sequence: Syntheticoligonucleotide
  source 1..20: mol_type = other DNA
gcagcaagcagcactctgcc

SEQ ID NO: 136 - DNA, 20 bp, synthetic construct
  misc_feature 1..20: note = Description of Artificial Sequence: Syntheticoligonucleotide
  source 1..20: mol_type = other DNA
gcttgggcccacgcaggggc

SEQ ID NO: 137 - DNA, 20 bp, synthetic construct
  misc_feature 1..20: note = Description of Artificial Sequence: Syntheticoligonucleotide
  source 1..20: mol_type = other DNA
gcttgggcccacgcaggggc

SEQ ID NO: 138 - DNA, 20 bp, synthetic construct
  misc_feature 1..20: note = Description of Artificial Sequence: Syntheticoligonucleotide
  source 1..20: mol_type = other DNA
gcttcgtggcaatgcgccac

SEQ ID NO: 139 - DNA, 20 bp, synthetic construct
  misc_feature 1..20: note = Description of Artificial Sequence: Syntheticoligonucleotide
  source 1..20: mol_type = other DNA
gcttgggcccacgcaggggc

SEQ ID NO: 140 - DNA, 20 bp, synthetic construct
  misc_feature 1..20: note = Description of Artificial Sequence: Syntheticoligonucleotide
  source 1..20: mol_type = other DNA
aagctggactctggccactc

SEQ ID NO: 141 - DNA, 20 bp, synthetic construct
  misc_feature 1..20: note = Description of Artificial Sequence: Syntheticoligonucleotide
  source 1..20: mol_type = other DNA
ttcttcttctgctcggactc

SEQ ID NO: 142 - DNA, 20 bp, synthetic construct
  misc_feature 1..20: note = Description of Artificial Sequence: Syntheticoligonucleotide
  source 1..20: mol_type = other DNA
ttcttcttctgctcggactc

SEQ ID NO: 143 - DNA, 20 bp, synthetic construct
  misc_feature 1..20: note = Description of Artificial Sequence: Syntheticoligonucleotide
  source 1..20: mol_type = other DNA
ttcttcttctgctcggactc

SEQ ID NO: 144 - DNA, 20 bp, synthetic construct
  misc_feature 1..20: note = Description of Artificial Sequence: Syntheticoligonucleotide
  source 1..20: mol_type = other DNA
gagtttctcatctgtgcccc

SEQ ID NO: 145 - DNA, 20 bp, synthetic construct
  misc_feature 1..20: note = Description of Artificial Sequence: Syntheticoligonucleotide
  source 1..20: mol_type = other DNA
ttcctcctccagcttctgcc

SEQ ID NO: 146 - DNA, 20 bp, synthetic construct
  misc_feature 1..20: note = Description of Artificial Sequence: Syntheticoligonucleotide
  source 1..20: mol_type = other DNA
ttcctcctccagcttctgcc

SEQ ID NO: 147 - DNA, 20 bp, synthetic construct
  misc_feature 1..20: note = Description of Artificial Sequence: Syntheticoligonucleotide
  source 1..20: mol_type = other DNA
agcagaagaagaagggctcc

SEQ ID NO: 148 - DNA, 20 bp, synthetic construct
  misc_feature 1..20: note = Description of Artificial Sequence: Syntheticoligonucleotide
  source 1..20: mol_type = other DNA
aagctggactctggccactc

SEQ ID NO: 149 - RNA, 20 nt, synthetic construct
  misc_feature 1..20: note = Description of Artificial Sequence: Syntheticoligonucleotide
  source 1..20: mol_type = other RNA
gtgtccgagcagaagaagaa

SEQ ID NO: 150 - RNA, 20 nt, synthetic construct
  misc_feature 1..20: note = Description of Artificial Sequence: Syntheticoligonucleotide
  source 1..20: mol_type = other RNA
gactccgagcagaagaagaa

SEQ ID NO: 151 - RNA, 20 nt, synthetic construct
  misc_feature 1..20: note = Description of Artificial Sequence: Syntheticoligonucleotide
  source 1..20: mol_type = other RNA
gagaccgagcagaagaagaa

SEQ ID NO: 152 - RNA, 20 nt, synthetic construct
  misc_feature 1..20: note = Description of Artificial Sequence: Syntheticoligonucleotide
  source 1..20: mol_type = other RNA
gagtgcgagcagaagaagaa

SEQ ID NO: 153 - RNA, 20 nt, synthetic construct
  misc_feature 1..20: note = Description of Artificial Sequence: Syntheticoligonucleotide
  source 1..20: mol_type = other RNA
gagtcggagcagaagaagaa

SEQ ID NO: 154 - RNA, 20 nt, synthetic construct
  misc_feature 1..20: note = Description of Artificial Sequence: Syntheticoligonucleotide
  source 1..20: mol_type = other RNA
gagtcccagcagaagaagaa

SEQ ID NO: 155 - RNA, 20 nt, synthetic construct
  misc_feature 1..20: note = Description of Artificial Sequence: Syntheticoligonucleotide
  source 1..20: mol_type = other RNA
gagtccgtgcagaagaagaa

SEQ ID NO: 156 - RNA, 20 nt, synthetic construct
  misc_feature 1..20: note = Description of Artificial Sequence: Syntheticoligonucleotide
  source 1..20: mol_type = other RNA
gagtccgaccagaagaagaa

SEQ ID NO: 157 - RNA, 20 nt, synthetic construct
  misc_feature 1..20: note = Description of Artificial Sequence: Syntheticoligonucleotide
  source 1..20: mol_type = other RNA
gagtccgaggagaagaagaa

SEQ ID NO: 158 - RNA, 20 nt, synthetic construct
  misc_feature 1..20: note = Description of Artificial Sequence: Syntheticoligonucleotide
  source 1..20: mol_type = other RNA
gagtccgagctgaagaagaa

SEQ ID NO: 159 - RNA, 20 nt, synthetic construct
  misc_feature 1..20: note = Description of Artificial Sequence: Syntheticoligonucleotide
  source 1..20: mol_type = other RNA
gtgtccgagcagaagaagaa

SEQ ID NO: 160 - RNA, 20 nt, synthetic construct
  misc_feature 1..20: note = Description of Artificial Sequence: Syntheticoligonucleotide
  source 1..20: mol_type = other RNA
gactccgagcagaagaagaa

SEQ ID NO: 161 - RNA, 20 nt, synthetic construct
  misc_feature 1..20: note = Description of Artificial Sequence: Syntheticoligonucleotide
  source 1..20: mol_type = other RNA
gagaccgagcagaagaagaa

SEQ ID NO: 162 - RNA, 20 nt, synthetic construct
  misc_feature 1..20: note = Description of Artificial Sequence: Syntheticoligonucleotide
  source 1..20: mol_type = other RNA
gagtgcgagcagaagaagaa

SEQ ID NO: 163 - RNA, 20 nt, synthetic construct
  misc_feature 1..20: note = Description of Artificial Sequence: Syntheticoligonucleotide
  source 1..20: mol_type = other RNA
gagtcggagcagaagaagaa

SEQ ID NO: 164 - RNA, 20 nt, synthetic construct
  misc_feature 1..20: note = Description of Artificial Sequence: Syntheticoligonucleotide
  source 1..20: mol_type = other RNA
gagtcccagcagaagaagaa

SEQ ID NO: 165 - RNA, 20 nt, synthetic construct
  misc_feature 1..20: note = Description of Artificial Sequence: Syntheticoligonucleotide
  source 1..20: mol_type = other RNA
gagtccgtgcagaagaagaa

SEQ ID NO: 166 - RNA, 20 nt, synthetic construct
  misc_feature 1..20: note = Description of Artificial Sequence: Syntheticoligonucleotide
  source 1..20: mol_type = other RNA
gagtccgaccagaagaagaa

SEQ ID NO: 167 - RNA, 20 nt, synthetic construct
  misc_feature 1..20: note = Description of Artificial Sequence: Syntheticoligonucleotide
  source 1..20: mol_type = other RNA
gagtccgaggagaagaagaa

SEQ ID NO: 168 - RNA, 20 nt, synthetic construct
  misc_feature 1..20: note = Description of Artificial Sequence: Syntheticoligonucleotide
  source 1..20: mol_type = other RNA
gagtccgagctgaagaagaa

SEQ ID NO: 169 - RNA, 20 nt, synthetic construct
  misc_feature 1..20: note = Description of Artificial Sequence: Syntheticoligonucleotide
  source 1..20: mol_type = other RNA
gacacctccaatgactaggg

SEQ ID NO: 170 - RNA, 20 nt, synthetic construct
  misc_feature 1..20: note = Description of Artificial Sequence: Syntheticoligonucleotide
  source 1..20: mol_type = other RNA
gtgacctccaatgactaggg

SEQ ID NO: 171 - RNA, 20 nt, synthetic construct
  misc_feature 1..20: note = Description of Artificial Sequence: Syntheticoligonucleotide
  source 1..20: mol_type = other RNA
gtctcctccaatgactaggg

SEQ ID NO: 172 - RNA, 20 nt, synthetic construct
  misc_feature 1..20: note = Description of Artificial Sequence: Syntheticoligonucleotide
  source 1..20: mol_type = other RNA
gtcagctccaatgactaggg

SEQ ID NO: 173 - RNA, 20 nt, synthetic construct
  misc_feature 1..20: note = Description of Artificial Sequence: Syntheticoligonucleotide
  source 1..20: mol_type = other RNA
gtcacgtccaatgactaggg

SEQ ID NO: 174 - RNA, 20 nt, synthetic construct
  misc_feature 1..20: note = Description of Artificial Sequence: Syntheticoligonucleotide
  source 1..20: mol_type = other RNA
gtcaccaccaatgactaggg

SEQ ID NO: 175 - RNA, 20 nt, synthetic construct
  misc_feature 1..20: note = Description of Artificial Sequence: Syntheticoligonucleotide
  source 1..20: mol_type = other RNA
gtcacctgcaatgactaggg

SEQ ID NO: 176 - RNA, 20 nt, synthetic construct
  misc_feature 1..20: note = Description of Artificial Sequence: Syntheticoligonucleotide
  source 1..20: mol_type = other RNA
gtcacctcgaatgactaggg

SEQ ID NO: 177 - RNA, 20 nt, synthetic construct
  misc_feature 1..20: note = Description of Artificial Sequence: Syntheticoligonucleotide
  source 1..20: mol_type = other RNA
gtcacctcctatgactaggg

SEQ ID NO: 178 - RNA, 20 nt, synthetic construct
  misc_feature 1..20: note = Description of Artificial Sequence: Syntheticoligonucleotide
  source 1..20: mol_type = other RNA
gtcacctccattgactaggg

SEQ ID NO: 179 - RNA, 20 nt, synthetic construct
  misc_feature 1..20: note = Description of Artificial Sequence: Syntheticoligonucleotide
  source 1..20: mol_type = other RNA
gtcatcgatgtcctccccat

SEQ ID NO: 180 - RNA, 20 nt, synthetic construct
  misc_feature 1..20: note = Description of Artificial Sequence: Syntheticoligonucleotide
  source 1..20: mol_type = other RNA
gagatcgatgtcctccccat

SEQ ID NO: 181 - RNA, 20 nt, synthetic construct
  misc_feature 1..20: note = Description of Artificial Sequence: Syntheticoligonucleotide
  source 1..20: mol_type = other RNA
gacttcgatgtcctccccat

SEQ ID NO: 182 - RNA, 20 nt, synthetic construct
  misc_feature 1..20: note = Description of Artificial Sequence: Syntheticoligonucleotide
  source 1..20: mol_type = other RNA
gacaacgatgtcctccccat

SEQ ID NO: 183 - RNA, 20 nt, synthetic construct
  misc_feature 1..20: note = Description of Artificial Sequence: Syntheticoligonucleotide
  source 1..20: mol_type = other RNA
gacatggatgtcctccccat

SEQ ID NO: 184 - RNA, 20 nt, synthetic construct
  misc_feature 1..20: note = Description of Artificial Sequence: Syntheticoligonucleotide
  source 1..20: mol_type = other RNA
gacatccatgtcctccccat

SEQ ID NO: 185 - RNA, 20 nt, synthetic construct
  misc_feature 1..20: note = Description of Artificial Sequence: Syntheticoligonucleotide
  source 1..20: mol_type = other RNA
gacatcgttgtcctccccat

SEQ ID NO: 186 - RNA, 20 nt, synthetic construct
  misc_feature 1..20: note = Description of Artificial Sequence: Syntheticoligonucleotide
  source 1..20: mol_type = other RNA
gacatcgaagtcctccccat

SEQ ID NO: 187 - RNA, 20 nt, synthetic construct
  misc_feature 1..20: note = Description of Artificial Sequence: Syntheticoligonucleotide
  source 1..20: mol_type = other RNA
gacatcgatctcctccccat

SEQ ID NO: 188 - RNA, 20 nt, synthetic construct
  misc_feature 1..20: note = Description of Artificial Sequence: Syntheticoligonucleotide
  source 1..20: mol_type = other RNA
gacatcgatgacctccccat

SEQ ID NO: 189 - RNA, 20 nt, synthetic construct
  misc_feature 1..20: note = Description of Artificial Sequence: Syntheticoligonucleotide
  source 1..20: mol_type = other RNA
gggccaccggttgatgtgat

SEQ ID NO: 190 - RNA, 20 nt, synthetic construct
  misc_feature 1..20: note = Description of Artificial Sequence: Syntheticoligonucleotide
  source 1..20: mol_type = other RNA
gccccaccggttgatgtgat

SEQ ID NO: 191 - RNA, 20 nt, synthetic construct
  misc_feature 1..20: note = Description of Artificial Sequence: Syntheticoligonucleotide
  source 1..20: mol_type = other RNA
gcggcaccggttgatgtgat

SEQ ID NO: 192 - RNA, 20 nt, synthetic construct
  misc_feature 1..20: note = Description of Artificial Sequence: Syntheticoligonucleotide
  source 1..20: mol_type = other RNA
gcgcgaccggttgatgtgat

SEQ ID NO: 193 - RNA, 20 nt, synthetic construct
  misc_feature 1..20: note = Description of Artificial Sequence: Syntheticoligonucleotide
  source 1..20: mol_type = other RNA
gcgcctccggttgatgtgat

SEQ ID NO: 194 - RNA, 20 nt, synthetic construct
  misc_feature 1..20: note = Description of Artificial Sequence: Syntheticoligonucleotide
  source 1..20: mol_type = other RNA
gcgccagcggttgatgtgat

SEQ ID NO: 195 - RNA, 20 nt, synthetic construct
  misc_feature 1..20: note = Description of Artificial Sequence: Syntheticoligonucleotide
  source 1..20: mol_type = other RNA
gcgccacgggttgatgtgat

SEQ ID NO: 196 - RNA, 20 nt, synthetic construct
  misc_feature 1..20: note = Description of Artificial Sequence: Syntheticoligonucleotide
  source 1..20: mol_type = other RNA
gcgccacccgttgatgtgat

SEQ ID NO: 197 - RNA, 20 nt, synthetic construct
  misc_feature 1..20: note = Description of Artificial Sequence: Syntheticoligonucleotide
  source 1..20: mol_type = other RNA
gcgccaccgcttgatgtgat

SEQ ID NO: 198 - RNA, 20 nt, synthetic construct
  misc_feature 1..20: note = Description of Artificial Sequence: Syntheticoligonucleotide
  source 1..20: mol_type = other RNA
gcgccaccggatgatgtgat

SEQ ID NO: 199 - RNA, 20 nt, synthetic construct
  misc_feature 1..20: note = Description of Artificial Sequence: Syntheticoligonucleotide
  source 1..20: mol_type = other RNA
gggccacagatgagaaactc

SEQ ID NO: 200 - RNA, 20 nt, synthetic construct
  misc_feature 1..20: note = Description of Artificial Sequence: Syntheticoligonucleotide
  source 1..20: mol_type = other RNA
gttcaaacggcagaagctgg

SEQ ID NO: 201 - RNA, 20 nt, synthetic construct
  misc_feature 1..20: note = Description of Artificial Sequence: Syntheticoligonucleotide
  source 1..20: mol_type = other RNA
gtactaacggcagaagctgg

SEQ ID NO: 202 - RNA, 20 nt, synthetic construct
  misc_feature 1..20: note = Description of Artificial Sequence: Syntheticoligonucleotide
  source 1..20: mol_type = other RNA
gtacaaacgggagaagctgg

SEQ ID NO: 203 - RNA, 20 nt, synthetic construct
  misc_feature 1..20: note = Description of Artificial Sequence: Syntheticoligonucleotide
  source 1..20: mol_type = other RNA
gccagaagctggaggaggaa

SEQ ID NO: 204 - RNA, 20 nt, synthetic construct
  misc_feature 1..20: note = Description of Artificial Sequence: Syntheticoligonucleotide
  source 1..20: mol_type = other RNA
ggcacaagctggaggaggaa

SEQ ID NO: 205 - RNA, 20 nt, synthetic construct
  misc_feature 1..20: note = Description of Artificial Sequence: Syntheticoligonucleotide
  source 1..20: mol_type = other RNA
ggcagaacctggaggaggaa

SEQ ID NO: 206 - RNA, 20 nt, synthetic construct
  misc_feature 1..20: note = Description of Artificial Sequence: Syntheticoligonucleotide
  source 1..20: mol_type = other RNA
ggcagaagcaggaggaggaa

SEQ ID NO: 207 - RNA, 20 nt, synthetic construct
  misc_feature 1..20: note = Description of Artificial Sequence: Syntheticoligonucleotide
  source 1..20: mol_type = other RNA
ggcagaagctcgaggaggaa

SEQ ID NO: 208 - RNA, 20 nt, synthetic construct
  misc_feature 1..20: note = Description of Artificial Sequence: Syntheticoligonucleotide
  source 1..20: mol_type = other RNA
gcacccatcacatcaaccgg

SEQ ID NO: 209 - RNA, 20 nt, synthetic construct
  misc_feature 1..20: note = Description of Artificial Sequence: Syntheticoligonucleotide
  source 1..20: mol_type = other RNA
gctcccttcacatcaaccgg

SEQ ID NO: 210 - RNA, 20 nt, synthetic construct
  misc_feature 1..20: note = Description of Artificial Sequence: Syntheticoligonucleotide
  source 1..20: mol_type = other RNA
gctcccaacacatcaaccgg

SEQ ID NO: 211 - RNA, 20 nt, synthetic construct
  misc_feature 1..20: note = Description of Artificial Sequence: Syntheticoligonucleotide
  source 1..20: mol_type = other RNA
gctcccatcagatcaaccgg

SEQ ID NO: 212 - RNA, 20 nt, synthetic construct
  misc_feature 1..20: note = Description of Artificial Sequence: Syntheticoligonucleotide
  source 1..20: mol_type = other RNA
ggcagtgtgctgcttgctgc

SEQ ID NO: 213 - RNA, 20 nt, synthetic construct
  misc_feature 1..20: note = Description of Artificial Sequence: Syntheticoligonucleotide
  source 1..20: mol_type = other RNA
ggcagagtgcagcttgctgc

SEQ ID NO: 214 - RNA, 20 nt, synthetic construct
  misc_feature 1..20: note = Description of Artificial Sequence: Syntheticoligonucleotide
  source 1..20: mol_type = other RNA
gccccagcgtgggcccaagc

SEQ ID NO: 215 - RNA, 20 nt, synthetic construct
  misc_feature 1..20: note = Description of Artificial Sequence: Syntheticoligonucleotide
  source 1..20: mol_type = other RNA
gcccctgcctgggcccaagc

SEQ ID NO: 216 - RNA, 20 nt, synthetic construct
  misc_feature 1..20: note = Description of Artificial Sequence: Syntheticoligonucleotide
  source 1..20: mol_type = other RNA
gtggcccattgccacgaagc

SEQ ID NO: 217 - RNA, 20 nt, synthetic construct
  misc_feature 1..20: note = Description of Artificial Sequence: Syntheticoligonucleotide
  source 1..20: mol_type = other RNA
gcccctgcgtcggcccaagc

SEQ ID NO: 218 - RNA, 20 nt, synthetic construct
  misc_feature 1..20: note = Description of Artificial Sequence: Syntheticoligonucleotide
  source 1..20: mol_type = other RNA
gagtggcctgagtccagctt

SEQ ID NO: 219 - RNA, 20 nt, synthetic construct
  misc_feature 1..20: note = Description of Artificial Sequence: Syntheticoligonucleotide
  source 1..20: mol_type = other RNA
gagaccgagcagaagaagaa

SEQ ID NO: 220 - RNA, 20 nt, synthetic construct
  misc_feature 1..20: note = Description of Artificial Sequence: Syntheticoligonucleotide
  source 1..20: mol_type = other RNA
gagtccgaggagaagaagaa

SEQ ID NO: 221 - RNA, 20 nt, synthetic construct
  misc_feature 1..20: note = Description of Artificial Sequence: Syntheticoligonucleotide
  source 1..20: mol_type = other RNA
gagtccgagctgaagaagaa

SEQ ID NO: 222 - RNA, 20 nt, synthetic construct
  misc_feature 1..20: note = Description of Artificial Sequence: Syntheticoligonucleotide
  source 1..20: mol_type = other RNA
ggggcacagttgagaaactc

SEQ ID NO: 223 - RNA, 20 nt, synthetic construct
  misc_feature 1..20: note = Description of Artificial Sequence: Syntheticoligonucleotide
  source 1..20: mol_type = other RNA
ggcagaaggtggaggaggaa

SEQ ID NO: 224 - RNA, 20 nt, synthetic construct
  misc_feature 1..20: note = Description of Artificial Sequence: Syntheticoligonucleotide
  source 1..20: mol_type = other RNA
ggcagaagcaggaggaggaa

SEQ ID NO: 225 - RNA, 20 nt, synthetic construct
  misc_feature 1..20: note = Description of Artificial Sequence: Syntheticoligonucleotide
  source 1..20: mol_type = other RNA
ggagcccttgttcttctgct

SEQ ID NO: 226 - RNA, 20 nt, synthetic construct
  misc_feature 1..20: note = Description of Artificial Sequence: Syntheticoligonucleotide
  source 1..20: mol_type = other RNA
gagtggcctgagtccagctt

SEQ ID NO: 227 - RNA, 20 nt, synthetic construct
  misc_feature 1..20: note = Description of Artificial Sequence: Syntheticoligonucleotide
  source 1..20: mol_type = other RNA
gacacctccaatgactaggg

SEQ ID NO: 228 - RNA, 20 nt, synthetic construct
  misc_feature 1..20: note = Description of Artificial Sequence: Syntheticoligonucleotide
  source 1..20: mol_type = other RNA
gtgacctccaatgactaggg

SEQ ID NO: 229 - RNA, 20 nt, synthetic construct
  misc_feature 1..20: note = Description of Artificial Sequence: Syntheticoligonucleotide
  source 1..20: mol_type = other RNA
gtctcctccaatgactaggg

SEQ ID NO: 230 - RNA, 20 nt, synthetic construct
  misc_feature 1..20: note = Description of Artificial Sequence: Syntheticoligonucleotide
  source 1..20: mol_type = other RNA
gtcagctccaatgactaggg

SEQ ID NO: 231 - RNA, 20 nt, synthetic construct
  misc_feature 1..20: note = Description of Artificial Sequence: Syntheticoligonucleotide
  source 1..20: mol_type = other RNA
gtcacgtccaatgactaggg

SEQ ID NO: 232 - RNA, 20 nt, synthetic construct
  misc_feature 1..20: note = Description of Artificial Sequence: Syntheticoligonucleotide
  source 1..20: mol_type = other RNA
gtcaccaccaatgactaggg

SEQ ID NO: 233 - RNA, 20 nt, synthetic construct
  misc_feature 1..20: note = Description of Artificial Sequence: Syntheticoligonucleotide
  source 1..20: mol_type = other RNA
gtcacctgcaatgactaggg

SEQ ID NO: 234 - RNA, 20 nt, synthetic construct
  misc_feature 1..20: note = Description of Artificial Sequence: Syntheticoligonucleotide
  source 1..20: mol_type = other RNA
gtcacctcgaatgactaggg

SEQ ID NO: 235 - RNA, 20 nt, synthetic construct
  misc_feature 1..20: note = Description of Artificial Sequence: Syntheticoligonucleotide
  source 1..20: mol_type = other RNA
gtcacctcctatgactaggg

SEQ ID NO: 236 - RNA, 20 nt, synthetic construct
  misc_feature 1..20: note = Description of Artificial Sequence: Syntheticoligonucleotide
  source 1..20: mol_type = other RNA
gtcacctccattgactaggg

SEQ ID NO: 237 - RNA, 20 nt, synthetic construct
  misc_feature 1..20: note = Description of Artificial Sequence: Syntheticoligonucleotide
  source 1..20: mol_type = other RNA
gtcatcgatgtcctccccat

SEQ ID NO: 238 - RNA, 20 nt, synthetic construct
  misc_feature 1..20: note = Description of Artificial Sequence: Syntheticoligonucleotide
  source 1..20: mol_type = other RNA
gagatcgatgtcctccccat

SEQ ID NO: 239 - RNA, 20 nt, synthetic construct
  misc_feature 1..20: note = Description of Artificial Sequence: Syntheticoligonucleotide
  source 1..20: mol_type = other RNA
gacttcgatgtcctccccat

SEQ ID NO: 240 - RNA, 20 nt, synthetic construct
  misc_feature 1..20: note = Description of Artificial Sequence: Syntheticoligonucleotide
  source 1..20: mol_type = other RNA
gacaacgatgtcctccccat

SEQ ID NO: 241 - RNA, 20 nt, synthetic construct
  misc_feature 1..20: note = Description of Artificial Sequence: Syntheticoligonucleotide
  source 1..20: mol_type = other RNA
gacatggatgtcctccccat

SEQ ID NO: 242 - RNA, 20 nt, synthetic construct
  misc_feature 1..20: note = Description of Artificial Sequence: Syntheticoligonucleotide
  source 1..20: mol_type = other RNA
gacatccatgtcctccccat

SEQ ID NO: 243 - RNA, 20 nt, synthetic construct
  misc_feature 1..20: note = Description of Artificial Sequence: Syntheticoligonucleotide
  source 1..20: mol_type = other RNA
gacatcgttgtcctccccat

SEQ ID NO: 244 - RNA, 20 nt, synthetic construct
  misc_feature 1..20: note = Description of Artificial Sequence: Syntheticoligonucleotide
  source 1..20: mol_type = other RNA
gacatcgaagtcctccccat

SEQ ID NO: 245 - RNA, 20 nt, synthetic construct
  misc_feature 1..20: note = Description of Artificial Sequence: Syntheticoligonucleotide
  source 1..20: mol_type = other RNA
gacatcgatctcctccccat

SEQ ID NO: 246 - RNA, 20 nt, synthetic construct
  misc_feature 1..20: note = Description of Artificial Sequence: Syntheticoligonucleotide
  source 1..20: mol_type = other RNA
gacatcgatgacctccccat

SEQ ID NO: 247 - RNA, 20 nt, synthetic construct
  misc_feature 1..20: note = Description of Artificial Sequence: Syntheticoligonucleotide
  source 1..20: mol_type = other RNA
gggccaccggttgatgtgat

SEQ ID NO: 248 - RNA, 20 nt, synthetic construct
  misc_feature 1..20: note = Description of Artificial Sequence: Syntheticoligonucleotide
  source 1..20: mol_type = other RNA
gccccaccggttgatgtgat

SEQ ID NO: 249 - RNA, 20 nt, synthetic construct
  misc_feature 1..20: note = Description of Artificial Sequence: Syntheticoligonucleotide
  source 1..20: mol_type = other RNA
gcggcaccggttgatgtgat

SEQ ID NO: 250 - RNA, 20 nt, synthetic construct
  misc_feature 1..20: note = Description of Artificial Sequence: Syntheticoligonucleotide
  source 1..20: mol_type = other RNA
gcgcgaccggttgatgtgat

SEQ ID NO: 251 - RNA, 20 nt, synthetic construct
  misc_feature 1..20: note = Description of Artificial Sequence: Syntheticoligonucleotide
  source 1..20: mol_type = other RNA
gcgcctccggttgatgtgat

SEQ ID NO: 252 - RNA, 20 nt, synthetic construct
  misc_feature 1..20: note = Description of Artificial Sequence: Syntheticoligonucleotide
  source 1..20: mol_type = other RNA
gcgccagcggttgatgtgat

SEQ ID NO: 253 - RNA, 20 nt, synthetic construct
  misc_feature 1..20: note = Description of Artificial Sequence: Syntheticoligonucleotide
  source 1..20: mol_type = other RNA
gcgccacgggttgatgtgat

SEQ ID NO: 254 - RNA, 20 nt, synthetic construct
  misc_feature 1..20: note = Description of Artificial Sequence: Syntheticoligonucleotide
  source 1..20: mol_type = other RNA
gcgccacccgttgatgtgat

SEQ ID NO: 255 - RNA, 20 nt, synthetic construct
  misc_feature 1..20: note = Description of Artificial Sequence: Syntheticoligonucleotide
  source 1..20: mol_type = other RNA
gcgccaccgcttgatgtgat

SEQ ID NO: 256 - RNA, 20 nt, synthetic construct
  misc_feature 1..20: note = Description of Artificial Sequence: Syntheticoligonucleotide
  source 1..20: mol_type = other RNA
gcgccaccggatgatgtgat

SEQ ID NO: 257 - RNA, 20 nt, synthetic construct
  misc_feature 1..20: note = Description of Artificial Sequence: Syntheticoligonucleotide
  source 1..20: mol_type = other RNA
gggccacagatgagaaactc

SEQ ID NO: 258 - RNA, 20 nt, synthetic construct
  misc_feature 1..20: note = Description of Artificial Sequence: Syntheticoligonucleotide
  source 1..20: mol_type = other RNA
gttcaaacggcagaagctgg

SEQ ID NO: 259 - RNA, 20 nt, synthetic construct
  misc_feature 1..20: note = Description of Artificial Sequence: Syntheticoligonucleotide
  source 1..20: mol_type = other RNA
gtactaacggcagaagctgg

SEQ ID NO: 260 - RNA, 20 nt, synthetic construct
  misc_feature 1..20: note = Description of Artificial Sequence: Syntheticoligonucleotide
  source 1..20: mol_type = other RNA
gtacaaacgggagaagctgg

SEQ ID NO: 261 - RNA, 20 nt, synthetic construct
  misc_feature 1..20: note = Description of Artificial Sequence: Syntheticoligonucleotide
  source 1..20: mol_type = other RNA
gccagaagctggaggaggaa

SEQ ID NO: 262 - RNA, 20 nt, synthetic construct
  misc_feature 1..20: note = Description of Artificial Sequence: Syntheticoligonucleotide
  source 1..20: mol_type = other RNA
ggcacaagctggaggaggaa

SEQ ID NO: 263 - RNA, 20 nt, synthetic construct
  misc_feature 1..20: note = Description of Artificial Sequence: Syntheticoligonucleotide
  source 1..20: mol_type = other RNA
ggcagaacctggaggaggaa

SEQ ID NO: 264 - RNA, 20 nt, synthetic construct
  misc_feature 1..20: note = Description of Artificial Sequence: Syntheticoligonucleotide
  source 1..20: mol_type = other RNA
ggcagaagcaggaggaggaa

SEQ ID NO: 265 - RNA, 20 nt, synthetic construct
  misc_feature 1..20: note = Description of Artificial Sequence: Syntheticoligonucleotide
  source 1..20: mol_type = other RNA
ggcagaagctcgaggaggaa

SEQ ID NO: 266 - RNA, 20 nt, synthetic construct
  misc_feature 1..20: note = Description of Artificial Sequence: Syntheticoligonucleotide
  source 1..20: mol_type = other RNA
gcacccatcacatcaaccgg

SEQ ID NO: 267 - RNA, 20 nt, synthetic construct
  misc_feature 1..20: note = Description of Artificial Sequence: Syntheticoligonucleotide
  source 1..20: mol_type = other RNA
gctcccttcacatcaaccgg

SEQ ID NO: 268 - RNA, 20 nt, synthetic construct
  misc_feature 1..20: note = Description of Artificial Sequence: Syntheticoligonucleotide
  source 1..20: mol_type = other RNA
gctcccaacacatcaaccgg

SEQ ID NO: 269 - RNA, 20 nt, synthetic construct
  misc_feature 1..20: note = Description of Artificial Sequence: Syntheticoligonucleotide
  source 1..20: mol_type = other RNA
gctcccatcagatcaaccgg

SEQ ID NO: 270 - RNA, 20 nt, synthetic construct
  misc_feature 1..20: note = Description of Artificial Sequence: Syntheticoligonucleotide
  source 1..20: mol_type = other RNA
ggcagtgtgctgcttgctgc

SEQ ID NO: 271 - RNA, 20 nt, synthetic construct
  misc_feature 1..20: note = Description of Artificial Sequence: Syntheticoligonucleotide
  source 1..20: mol_type = other RNA
ggcagagtgcagcttgctgc

SEQ ID NO: 272 - RNA, 20 nt, synthetic construct
  misc_feature 1..20: note = Description of Artificial Sequence: Syntheticoligonucleotide
  source 1..20: mol_type = other RNA
gccccagcgtgggcccaagc

SEQ ID NO: 273 - RNA, 20 nt, synthetic construct
  misc_feature 1..20: note = Description of Artificial Sequence: Syntheticoligonucleotide
  source 1..20: mol_type = other RNA
gcccctgcctgggcccaagc

SEQ ID NO: 274 - RNA, 20 nt, synthetic construct
  misc_feature 1..20: note = Description of Artificial Sequence: Syntheticoligonucleotide
  source 1..20: mol_type = other RNA
gtggcccattgccacgaagc

SEQ ID NO: 275 - RNA, 20 nt, synthetic construct
  misc_feature 1..20: note = Description of Artificial Sequence: Syntheticoligonucleotide
  source 1..20: mol_type = other RNA
gcccctgcgtcggcccaagc

SEQ ID NO: 276 - RNA, 20 nt, synthetic construct
  misc_feature 1..20: note = Description of Artificial Sequence: Syntheticoligonucleotide
  source 1..20: mol_type = other RNA
gagtggcctgagtccagctt

SEQ ID NO: 277 - RNA, 20 nt, synthetic construct
  misc_feature 1..20: note = Description of Artificial Sequence: Syntheticoligonucleotide
  source 1..20: mol_type = other RNA
gagaccgagcagaagaagaa

SEQ ID NO: 278 - RNA, 20 nt, synthetic construct
  misc_feature 1..20: note = Description of Artificial Sequence: Syntheticoligonucleotide
  source 1..20: mol_type = other RNA
gagtccgaggagaagaagaa

SEQ ID NO: 279 - RNA, 20 nt, synthetic construct
  misc_feature 1..20: note = Description of Artificial Sequence: Syntheticoligonucleotide
  source 1..20: mol_type = other RNA
gagtccgagctgaagaagaa

SEQ ID NO: 280 - RNA, 20 nt, synthetic construct
  misc_feature 1..20: note = Description of Artificial Sequence: Syntheticoligonucleotide
  source 1..20: mol_type = other RNA
ggggcacagttgagaaactc

SEQ ID NO: 281 - RNA, 20 nt, synthetic construct
  misc_feature 1..20: note = Description of Artificial Sequence: Syntheticoligonucleotide
  source 1..20: mol_type = other RNA
ggcagaaggtggaggaggaa

SEQ ID NO: 282 - RNA, 20 nt, synthetic construct
  misc_feature 1..20: note = Description of Artificial Sequence: Syntheticoligonucleotide
  source 1..20: mol_type = other RNA
ggcagaagcaggaggaggaa

SEQ ID NO: 283 - RNA, 20 nt, synthetic construct
  misc_feature 1..20: note = Description of Artificial Sequence: Syntheticoligonucleotide
  source 1..20: mol_type = other RNA
ggagcccttgttcttctgct

SEQ ID NO: 284 - RNA, 20 nt, synthetic construct
  misc_feature 1..20: note = Description of Artificial Sequence: Syntheticoligonucleotide
  source 1..20: mol_type = other RNA
gagtggcctgagtccagctt

SEQ ID NO: 285 - DNA, 24 bp, synthetic construct
  misc_feature 1..24: note = Description of Artificial Sequence: Syntheticoligonucleotide
  source 1..24: mol_type = other DNA
gagttcctactcagactgttactc

SEQ ID NO: 286 - DNA, 26 bp, synthetic construct
  misc_feature 1..26: note = Description of Artificial Sequence: Syntheticoligonucleotide
  source 1..26: mol_type = other DNA
gtgagttcctactcagactgttactc

SEQ ID NO: 287 - DNA, 28 bp, synthetic construct
  misc_feature 1..28: note = Description of Artificial Sequence: Syntheticoligonucleotide
  source 1..28: mol_type = other DNA
gtctgagttcctactcagactgttactc

SEQ ID NO: 288 - DNA, 24 bp, synthetic construct
  misc_feature 1..24: note = Description of Artificial Sequence: Syntheticoligonucleotide
  source 1..24: mol_type = other DNA
gtattcgtactcagactgttactc

SEQ ID NO: 289 - DNA, 26 bp, synthetic construct
  misc_feature 1..26: note = Description of Artificial Sequence: Syntheticoligonucleotide
  source 1..26: mol_type = other DNA
gagtattcgtactcagactgttactc

SEQ ID NO: 290 - DNA, 25 bp, synthetic construct
  misc_feature 1..25: note = Description of Artificial Sequence: Syntheticoligonucleotide
  source 1..25: mol_type = other DNA
gacttcggtccgagcagaagaagaa

SEQ ID NO: 291 - DNA, 26 bp, synthetic construct
  misc_feature 1..26: note = Description of Artificial Sequence: Syntheticoligonucleotide
  source 1..26: mol_type = other DNA
ggacttcggtccgagcagaagaagaa

SEQ ID NO: 292 - DNA, 28 bp, synthetic construct
  misc_feature 1..28: note = Description of Artificial Sequence: Syntheticoligonucleotide
  source 1..28: mol_type = other DNA
gcggacttcggtccgagcagaagaagaa

SEQ ID NO: 293 - DNA, 24 bp, synthetic construct
  misc_feature 1..24: note = Description of Artificial Sequence: Syntheticoligonucleotide
  source 1..24: mol_type = other DNA
gcgggagtccgagcagaagaagaa

SEQ ID NO: 294 - DNA, 25 bp, synthetic construct
  misc_feature 1..25: note = Description of Artificial Sequence: Syntheticoligonucleotide
  source 1..25: mol_type = other DNA
gtcgggagtccgagcagaagaagaa

SEQ ID NO: 295 - DNA, 26 bp, synthetic construct
  misc_feature 1..26: note = Description of Artificial Sequence: Syntheticoligonucleotide
  source 1..26: mol_type = other DNA
gctcgggagtccgagcagaagaagaa

SEQ ID NO: 296 - DNA, 30 bp, synthetic construct
  misc_feature 1..30: note = Description of Artificial Sequence: Syntheticoligonucleotide
  source 1..30: mol_type = other DNA
gttcacttcggggtggggggagtttgctcc

SEQ ID NO: 297 - DNA, 29 bp, synthetic construct
  misc_feature 1..29: note = Description of Artificial Sequence: Syntheticoligonucleotide
  source 1..29: mol_type = other DNA
gttcattcggggtggggggagtttgctcc

SEQ ID NO: 298 - DNA, 28 bp, synthetic construct
  misc_feature 1..28: note = Description of Artificial Sequence: Syntheticoligonucleotide
  source 1..28: mol_type = other DNA
gtccttcggggtggggggagtttgctcc

SEQ ID NO: 299 - DNA, 30 bp, synthetic construct
  misc_feature 1..30: note = Description of Artificial Sequence: Syntheticoligonucleotide
  source 1..30: mol_type = other DNA
gcttccttcggggtggggggagtttgctcc

SEQ ID NO: 300 - DNA, 30 bp, synthetic construct
  misc_feature 1..30: note = Description of Artificial Sequence: Syntheticoligonucleotide
  source 1..30: mol_type = other DNA
gtttccttcggggtggggggagtttgctcc

SEQ ID NO: 301 - DNA, 29 bp, synthetic construct
  misc_feature 1..29: note = Description of Artificial Sequence: Syntheticoligonucleotide
  source 1..29: mol_type = other DNA
gctccttcggggtggggggagtttgctcc

SEQ ID NO: 302 - DNA, 30 bp, synthetic construct
  misc_feature 1..30: note = Description of Artificial Sequence: Syntheticoligonucleotide
  source 1..30: mol_type = other DNA
gcccacttcggggtggggggagtttgctcc

SEQ ID NO: 303 - DNA, 29 bp, synthetic construct
  misc_feature 1..29: note = Description of Artificial Sequence: Syntheticoligonucleotide
  source 1..29: mol_type = other DNA
gcccattcggggtggggggagtttgctcc

SEQ ID NO: 304 - DNA, 29 bp, synthetic construct
  misc_feature 1..29: note = Description of Artificial Sequence: Syntheticoligonucleotide
  source 1..29: mol_type = other DNA
gccccttcggggtggggggagtttgctcc

SEQ ID NO: 305 - DNA, 30 bp, synthetic construct
  misc_feature 1..30: note = Description of Artificial Sequence: Syntheticoligonucleotide
  source 1..30: mol_type = other DNA
gcatccttcggtgtggggggagtttgctcc

SEQ ID NO: 306 - DNA, 25 bp, synthetic construct
  misc_feature 1..25: note = Description of Artificial Sequence: Syntheticoligonucleotide
  source 1..25: mol_type = other DNA
gccccgggtggggggagtttgctcc

SEQ ID NO: 307 - DNA, 24 bp, synthetic construct
  misc_feature 1..24: note = Description of Artificial Sequence: Syntheticoligonucleotide
  source 1..24: mol_type = other DNA
gcccgggtggggggagtttgctcc

SEQ ID NO: 308 - DNA, 23 bp, synthetic construct
  misc_feature 1..23: note = Description of Artificial Sequence: Syntheticoligonucleotide
  source 1..23: mol_type = other DNA
gccgggtggggggagtttgctcc

SEQ ID NO: 309 - DNA, 29 bp, synthetic construct
  misc_feature 1..29: note = Description of Artificial Sequence: Syntheticoligonucleotide
  source 1..29: mol_type = other DNA
gcacgttcgggtgagtgagtgtgtgcgtg

SEQ ID NO: 310 - DNA, 29 bp, synthetic construct
  misc_feature 1..29: note = Description of Artificial Sequence: Syntheticoligonucleotide
  source 1..29: mol_type = other DNA
gtacgttcgggtgagtgagtgtgtgcgtg

SEQ ID NO: 311 - DNA, 29 bp, synthetic construct
  misc_feature 1..29: note = Description of Artificial Sequence: Syntheticoligonucleotide
  source 1..29: mol_type = other DNA
gcatgttcgggtgagtgagtgtgtgcgtg

SEQ ID NO: 312 - DNA, 29 bp, synthetic construct
  misc_feature 1..29: note = Description of Artificial Sequence: Syntheticoligonucleotide
  source 1..29: mol_type = other DNA
gtatgttcgggtgagtgagtgtgtgcgtg

SEQ ID NO: 313 - DNA, 29 bp, synthetic construct
  misc_feature 1..29: note = Description of Artificial Sequence: Syntheticoligonucleotide
  source 1..29: mol_type = other DNA
gcgcgttcgggtgagtgagtgtgtgcgtg

SEQ ID NO: 314 - DNA, 29 bp, synthetic construct
  misc_feature 1..29: note = Description of Artificial Sequence: Syntheticoligonucleotide
  source 1..29: mol_type = other DNA
gcgtgttcgggtgagtgagtgtgtgcgtg

SEQ ID NO: 315 - DNA, 28 bp, synthetic construct
  misc_feature 1..28: note = Description of Artificial Sequence: Syntheticoligonucleotide
  source 1..28: mol_type = other DNA
gtaggttcgcctactcagactgttactc

SEQ ID NO: 316 - DNA, 21 bp, synthetic construct
  misc_feature 1..21: note = Description of Artificial Sequence: Syntheticoligonucleotide
  source 1..21: mol_type = other DNA
ggcctccccaaagcctggcca

SEQ ID NO: 317 - DNA, 21 bp, synthetic construct
  misc_feature 1..21: note = Description of Artificial Sequence: Syntheticoligonucleotide
  source 1..21: mol_type = other DNA
gacctccccatagcctggcca

SEQ ID NO: 318-319 - skipped (2 entries)

SEQ ID NO: 320 - DNA, 27 bp, synthetic construct
  misc_feature 1..27: note = Description of Artificial Sequence: Syntheticoligonucleotide
  source 1..27: mol_type = other DNA
tttcctgatggtccatgtctgttactc

SEQ ID NO: 321 - DNA, 27 bp, synthetic construct
  misc_feature 1..27: note = Description of Artificial Sequence: Syntheticoligonucleotide
  source 1..27: mol_type = other DNA
tttcgtgatggtccatgtctgttactc

SEQ ID NO: 322 - DNA, 27 bp, synthetic construct
  misc_feature 1..27: note = Description of Artificial Sequence: Syntheticoligonucleotide
  source 1..27: mol_type = other DNA
tttccagttggtccatgtctgttactc

SEQ ID NO: 323 - DNA, 27 bp, synthetic construct
  misc_feature 1..27: note = Description of Artificial Sequence: Syntheticoligonucleotide
  source 1..27: mol_type = other DNA
tttcctgatggtccatgtctgttactg

SEQ ID NO: 324 - DNA, 20 bp, synthetic construct
  misc_feature 1..20: note = Description of Artificial Sequence: Syntheticprimer
  source 1..20: mol_type = other DNA
ctgggactcaggcgggtcac

SEQ ID NO: 325 - DNA, 25 bp, synthetic construct
  misc_feature 1..25: note = Description of Artificial Sequence: Syntheticprimer
  source 1..25: mol_type = other DNA
cctcacacaacagcttcatgtcagc

SEQ ID NO: 326 - DNA, 20 bp, synthetic construct
  misc_feature 1..20: note = Description of Artificial Sequence: Syntheticoligonucleotide
  source 1..20: mol_type = other DNA
ctgatggtgcatgtctgtta

SEQ ID NO: 327 - DNA, 17 bp, synthetic construct
  misc_feature 1..17: note = Description of Artificial Sequence: Syntheticoligonucleotide
  source 1..17: mol_type = other DNA
ctgatggtgcatgtctg

SEQ ID NO: 328 - DNA, 32 bp, synthetic construct
  misc_feature 1..32: note = Description of Artificial Sequence: Syntheticoligonucleotide
  source 1..32: mol_type = other DNA
ctgatggtgcatgtctgttaagacatgcacca

SEQ ID NO: 329 - DNA, 26 bp, synthetic construct
  misc_feature 1..26: note = Description of Artificial Sequence: Syntheticoligonucleotide
  source 1..26: mol_type = other DNA
ctgatggtgcatgtctgcatgcacca

SEQ ID NO: 330 - DNA, 28 bp, unidentified
  misc_feature 1..28: note = Description of Unknown:DNMT1 oligonucleotide
  source 1..28: mol_type = genomic DNA
tttcctgatgggtccatgtctgttactc

SEQ ID NO: 331 - DNA, 20 bp, synthetic construct
  misc_feature 1..20: note = Description of Artificial Sequence: Syntheticoligonucleotide
  source 1..20: mol_type = other DNA
ctgatggtgcatgtctgtta

SEQ ID NO: 332 - DNA, 17 bp, synthetic construct
  misc_feature 1..17: note = Description of Artificial Sequence: Syntheticoligonucleotide
  source 1..17: mol_type = other DNA
ctgatggtgcatgtctg

SEQ ID NO: 333 - DNA, 32 bp, synthetic construct; identical to SEQ ID NO: 328
  misc_feature 1..32: note = Description of Artificial Sequence: Syntheticoligonucleotide
  source 1..32: mol_type = other DNA

SEQ ID NO: 334 - DNA, 26 bp, synthetic construct
  misc_feature 1..26: note = Description of Artificial Sequence: Syntheticoligonucleotide
  source 1..26: mol_type = other DNA
ctgatggtgcatgtctgcatgcacca

SEQ ID NO: 335 - DNA, 32 bp, synthetic construct
  misc_feature 1..32: note = Description of Artificial Sequence: Syntheticoligonucleotide
  source 1..32: mol_type = other DNA
gtgagtaggttcgcctactcagactgttactc

SEQ ID NO: 336 - DNA, 20 bp, synthetic construct
  misc_feature 1..20: note = Description of Artificial Sequence: Syntheticoligonucleotide
  source 1..20: mol_type = other DNA
atcctgtccctagtggcccc

SEQ ID NO: 337 - DNA, 20 bp, synthetic construct
  misc_feature 1..20: note = Description of Artificial Sequence: Syntheticoligonucleotide
  source 1..20: mol_type = other DNA
ggggccactagggacaggat

SEQ ID NO: 338 - RNA, 20 nt, synthetic construct
  misc_feature 1..20: note = Description of Artificial Sequence: Syntheticoligonucleotide
  source 1..20: mol_type = other RNA
ggggccactagggacaggat

SEQ ID NO: 339 - RNA, 18 nt, synthetic construct
  misc_feature 1..18: note = Description of Artificial Sequence: Syntheticoligonucleotide
  source 1..18: mol_type = other RNA
ggccactagggacaggat

SEQ ID NO: 340 - DNA, 20 bp, unidentified
  misc_feature 1..20: note = Description of Unknown:VEGFA1 target site oligonucleotide
  source 1..20: mol_type = genomic DNA
gggtggggggagtttgctcc

SEQ ID NO: 341 - DNA, 20 bp, unidentified
  misc_feature 1..20: note = Description of Unknown:VEGFA1 off-target site oligonucleotide
  source 1..20: mol_type = other DNA
ggatggagggagtttgctcc

SEQ ID NO: 342 - protein, 6 aa, synthetic construct
  REGION 1..6: note = Description of Artificial Sequence: Synthetic6xHis tag
HHHHHH

SEQ ID NO: 343 - DNA, 20 bp, synthetic construct
  misc_feature 1..20: note = Description of Artificial Sequence: Syntheticprimer
  misc_feature 1..20: note = 5'-Biotinylation
  source 1..20: mol_type = other DNA
ccaggatcagtgaaacgcac

SEQ ID NO: 344 - DNA, 20 bp, synthetic construct
  misc_feature 1..20: note = Description of Artificial Sequence: Syntheticprimer
  source 1..20: mol_type = other DNA
gagctctactggcttctgcg

SEQ ID NO: 345 - DNA, 17 bp, synthetic construct
  misc_feature 1..17: note = Description of Artificial Sequence: Syntheticprimer
  misc_feature 1..17: note = 5'-Biotinylation
  source 1..17: mol_type = other DNA
catgacgtgcagcaagc

SEQ ID NO: 346 - DNA, 17 bp, synthetic construct
  misc_feature 1..17: note = Description of Artificial Sequence: Syntheticprimer
  source 1..17: mol_type = other DNA
cgacgatgcgctgaatc

SEQ ID NO: 347 - DNA, 23 bp, synthetic construct
  misc_feature 1..23: note = Description of Artificial Sequence: Syntheticprimer
  misc_feature 1..23: note = 5'-Biotinylation
  source 1..23: mol_type = other DNA
gacctgcaggcatgcaagcttgg

SEQ ID NO: 348 - DNA, 22 bp, synthetic construct
  misc_feature 1..22: note = Description of Artificial Sequence: Syntheticprimer
  source 1..22: mol_type = other DNA
cagcgtccccggttgtgaatct